European Patent Application EP 4 141 113 A1, published March 1, 2023. Title: PAENIBACILLUS SP. MANNANASES. Applicant: Danisco US Inc. Application EP Div of EP16801909.9. The sequence listing filed with the application follows.

SEQUENCE LISTING (162 sequences)

SEQ ID NO: 1 - DNA, 984 bp, artificial sequence
  PspMan138 gene seq
gtgagaagcaaaaaattgtggatcagcttgttgtttgcgttaacgttaatctttacgatggcgttcagcaacatgtctgcgcaggctatggcgacaggcttttatgtttcaggcaacaaactgtatgatagcacaggcaaagagtttgttatgagaggcgttaatcatggccatacctggtttaaaaacgatctgaatgaggcgattccggctattgcaaaaacaggcgcaaatacagttagaattgttctgtcaaatggcgtgcagtatacgagagatgatctggacgcagtcaaaaacatcatcaatgtcgtcaaccagaacaaaatgatagcagttctggaagttcatgatgcaacgggcaaagatgattacgattcactggatgcagcaatcaactattggatctcaattaaagaagcgctgatcggcaaagaagatcgcgttattgttaatattgcgaacgaatggatgggcacatggaatggctcagcatgggcagatggctacaaaaaagcaattccgaaactgagaaatgcaggcatcaaaaacacactgattgttgatgcggcaggctggggacaatatccgcaatcaattgttgattatggccaaagcgtttttgcagcagatagcttaaaaaatacagtctttagcatccatatgtacgaatacgctggaaaggatgcagcaacagttaaagcgaatatggaaaacgtcctgaataaaggcctggcactgattattggcgaatttggctgctatcatgtgaatggcgacgttgatgaactggcgattatgagatatggccaagaattgggcgttggctggcttgcatggtcatggtatggaaattcagacggccttcggtatctggatatggcaacaggaccgaatggatcactgacatcatttggcaatacagtcgtcaatgatacgtatggaatcaaaaatacgagccagaaagctggcatctttcagtaa

SEQ ID NO: 2 - DNA, 608 bp, Bacillus subtilis
gaattctccattttcttctgctatcaaaataacagactcgtgattttccaaacgagctttcaaaaaagcctctgccccttgcaaatcggatgcctgtctataaaattcccgatattggttaaacagcggcgcaatggcggccgcatctgatgtctttgcttggcgaatgttcatcttatttcttcctccctctcaataattttttcattctatcccttttctgtaaagtttatttttcagaatacttttatcatcatgctttgaaaaaatatcacgataatatccattgttctcacggaagcacacgcaggtcatttgaacgaattttttcgacaggaatttgccgggactcaggagcatttaacctaaaaaagcatgacatttcagcataatgaacatttactcatgtctattttcgttcttttctgtatgaaaatagttatttcgagtctctacggaaatagcgagagatgatatacctaaatagagataaaatcatctcaaaaaaatgggtctactaaaatattattccatctattacaataaattcacagaatagtcttttaagtaagtctactctgaatttttttaaaaggagagggtaaaga

SEQ ID NO: 3 - DNA, 87 bp, Bacillus subtilis
gtgagaagcaaaaaattgtggatcagcttgttgtttgcgttaacgttaatctttacgatggcgttcagcaacatgtctgctagcgca

SEQ ID NO: 4 - protein, 29 aa, Bacillus subtilis
VRSKKLWISLLFALTLIFTMAFSNMSAQA

SEQ ID NO: 5 - DNA, 93 bp, artificial sequence
  terminator
ggttaccttgaatgtatataaacattctcaaagggatttctaataaaaaacgctcggttgccgccgggcgttttttatgcatcgatggaattc

SEQ ID NO: 6 - DNA, 21 bp, artificial sequence
  linker
ggatcctgactgcctgagctt

SEQ ID NO: 7 - DNA, 1819 bp, artificial sequence
  synthetic construct
taatacataaaaaaccggccttggccccgccggttttttattatttttcttcctccgcatgttcaatccgctccataatcgacggatggctccctctgaaaattttaacgagaaacggcgggttgacccggctcagtcccgtaacggccaagtcctgaaacgtctcaatcgccgcttcccggtttccggtcagctcaatgccgtaacggtcggcggcgttttcctgataccgggagacggcattcgtaatcggatccttagtgacattagaaaaccgactgtaaaaagtacagtcggcattatctcatattataaaagccagtcattaggcctatctgacaattcctgaatagagttcataaacaatcctgcatgataaccatcacaaacagaatgatgtacctgtaaagatagcggtaaatatattgaattacctttattaatgaattttcctgctgtaataatgggtagaaggtaattactattattattgatatttaagttaaacccagtaaatgaagtccatggaataatagaaagagaaaaagcattttcaggtataggtgttttgggaaacaatttccccgaaccattatatttctctacatcagaaaggtataaatcataaaactctttgaagtcattctttacaggagtccaaataccagagaatgttttagatacaccatcaaaaattgtataaagtggctctaacttatcccaataacctaactctccgtcgctattgtaaccagttctaaaagctgtatttgagtttatcacccttgtcactaagaaaataaatgcagggtaaaatttatatccttcttgttttatgtttcggtataaaacactaatatcaatttctgtggttatactaaaagtcgtttgttggttcaaataatgattaaatatctcttttctcttccaattgtctaaatcaattttattaaagttcatttgatatgcctcctaaatttttatctaaagtgaatttaggaggcttacttgtctgctttcttcattagaatcaatccttttttaaaagtcaatattactgtaacataaatatatattttaaaaatatcccactttatccaattttcgtttgtgatagagctggggaattctccattttcttctgctatcaaaataacagactcgtgattttccaaacgagctttcaaaaaagcctctgccccttgcaaatcggatgcctgtctataaaattcccgatattggttaaacagcggcgcaatggcggccgcatctgatgtctttgcttggcgaatgttcatcttatttcttcctccctctcaataattttttcattctatcccttttctgtaaagtttatttttcagaatacttttatcatcatgctttgaaaaaatatcacgataatatccattgttctcacggaagcacacgcaggtcatttgaacgaattttttcgacaggaatttgccgggactcaggagcatttaacctaaaaaagcatgacatttcagcataatgaacatttactcatgtctattttcgttcttttctgtatgaaaatagttatttcgagtctctacggaaatagcgagagatgatatacctaaatagagataaaatcatctcaaaaaaatgggtctactaaaatattattccatctattacaataaattcacagaatagtcttttaagtaagtctactctgaatttttttaaaaggagagggtaaagagtgagaagcaaaaaattgtggatcagcttgttgtttgcgttaacgttaatctttacgatggcgttcagcaacatgtctgcgcaggct

SEQ ID NO: 8 - DNA, 25 bp, artificial sequence
  primer
gttcagcaacatgtctgcgcaggct

SEQ ID NO: 9 - DNA, 27 bp, artificial sequence
  primer
gggccaaggccggttttttatgtatta

SEQ ID NO: 10 - DNA, 28 bp, artificial sequence
  primer
taatacataaaaaaccggccttggcccc

SEQ ID NO: 11 - DNA, 25 bp, artificial sequence
  primer
agcctgcgcagacatgttgctgaac

SEQ ID NO: 12 - protein, 327 aa, artificial sequence
  PspMan138 precursor protein sequence
VRSKKLWISLLFALTLIFTMAFSNMSAQAMATGFYVSGNKLYDSTGKEFVMRGVNHGHTWFKNDLNEAIPAIAKTGANTVRIVLSNGVQYTRDDLDAVKNIINVVNQNKMIAVLEVHDATGKDDYDSLDAAINYWISIKEALIGKEDRVIVNIANEWMGTWNGSAWADGYKKAIPKLRNAGIKNTLIVDAAGWGQYPQSIVDYGQSVFAADSLKNTVFSIHMYEYAGKDAATVKANMENVLNKGLALIIGEFGCYHVNGDVDELAIMRYGQELGVGWLAWSWYGNSDGLRYLDMATGPNGSLTSFGNTVVNDTYGIKNTSQKAGIFQ

SEQ ID NO: 13 - protein, 298 aa, artificial sequence
  PspMan138 mature enzyme sequence
MATGFYVSGNKLYDSTGKEFVMRGVNHGHTWFKNDLNEAIPAIAKTGANTVRIVLSNGVQYTRDDLDAVKNIINVVNQNKMIAVLEVHDATGKDDYDSLDAAINYWISIKEALIGKEDRVIVNIANEWMGTWNGSAWADGYKKAIPKLRNAGIKNTLIVDAAGWGQYPQSIVDYGQSVFAADSLKNTVFSIHMYEYAGKDAATVKANMENVLNKGLALIIGEFGCYHVNGDVDELAIMRYGQELGVGWLAWSWYGNSDGLRYLDMATGPNGSLTSFGNTVVNDTYGIKNTSQKAGIFQ

SEQ ID NO: 14 - protein, 297 aa, artificial sequence
  PspMan4 mature protein sequence
MATGFYVSGNKLYDSTGKPFVMRGVNHGHSWFKNDLNTAIPAIAKTGANTVRIVLSNGSLYTKDDLNAVKNIINVVNQNKMIAVLEVHDATGKDDYNSLDAAVNYWISIKEALIGKEDRVIVNIANEWYGTWNGSAWADGYKKAIPKLRNAGIKNTLIVDAAGWGQFPQSIVDYGQSVFAADSQKNTVFSIHMYEYAGKDAATVKANMENVLNKGLALIIGEFGGYHTNGDVDEYAIMRYGQEKGVGWLAWSWYGNSSGLNYLDMATGPNGSLTSFGNTVVNDTYGIKNTSQKAGIF

SEQ ID NO: 15 - protein, 10 aa, artificial sequence
  motif
  MISC_FEATURE (2)..(2): X is F or Y
  MISC_FEATURE (7)..(8): X iis any amino acid
WXKNDLXXAI

SEQ ID NO: 16 - protein, 12 aa, artificial sequence
  motif
  MISC_FEATURE (3)..(5): X is any amino acid
  MISC_FEATURE (8)..(8): X is any amino acid
  MISC_FEATURE (10)..(10): X is any amino acid
LDXXXGPXGXLT

SEQ ID NO: 17 - protein, 12 aa, artificial sequence
  motif
  MISC_FEATURE (3)..(3): X is M or L
  MISC_FEATURE (4)..(4): X is V or A
  MISC_FEATURE (5)..(5): X is A or T
  MISC_FEATURE (8)..(8): X is N, A or S
  MISC_FEATURE (10)..(10): X is S, T or N
LDXXXGPXGXLT

SEQ ID NO: 18 - protein, 12 aa, artificial sequence
  motif
  MISC_FEATURE (3)..(3): X is L or M
  MISC_FEATURE (8)..(8): X is N or A
  MISC_FEATURE (10)..(10): X is S or T
LDXATGPXGXLT

SEQ ID NO: 19 - protein, 297 aa, unknown
  Paenibacillus sp.
AATGFYVSGNKLYDSTGKAFVMRGVNHGHSWFKNDLNTAIPAIAKTGANTVRIVLSNGSLYTKDDLNAVKNIINVVNQNKMIAVLEVHDATGKDDYNSLDAAVNYWISIKEALIGKEDRVIVNIANEWYGTWNGSAWADGYKKAIPKLRNAGIKNTLIVDAAGWGQFPQSIVDYGQSVFAADSQKNTVFSIHMYEYAGKDAATVKANMENVLNKGLALIIGEFGGYHTNGDVDEYAIMRYGQEKGVGWLAWSWYGNSSGLNYLDMATGPNGSLTSFGNTVVNDTYGIKNTSQKAGIF

SEQ ID NO: 20 - protein, 296 aa, unknown
  Paenibacillus sp.
ATGFYVSGNKLYDSTGKAFVMRGVNHGHSWFKNDLNTAIPAIAKTGANTVRIVLSNGSLYTKDDLNAVKNIINVVNQNKMIAVLEVHDATGKEDYNSLDAAVNYWISIKEALIGKEDRVIVNIANEWYGTWNGSAWADGYKKAIPKLRNAGIKNTLIVDAAGWGQFPQSIVDYGQSVFAADSQKNTVFSIHMYEYAGKDAATVKANMENVLNKGLALIIGEFGGYHTNGDVDEYAIMRYGQEKGVGWLAWSWYGNSSGLNYLDMATGPNGSLTSFGNTVVNDTYGIKNTSQKAGIF

SEQ ID NO: 21 - protein, 297 aa, unknown
  Paenibacillus sp.
AATGFYVSGGKLYDSTGKAFVMRGVNHGHSWFKNDLNTAIPAIAKTGANTVRIVLSNGVQYTKDDLNAVKNIINVVSANKMIAVLEVHDATGKDDYNSLDAAVNYWISIKEALIGKEDRVIVNIANEWYGTWNGSAWADGYKKAIPKLRNAGINNTLIVDAAGWGQYPQSIVDYGQSVFAADSQKNTVFSIHMYEYAGKDAATVKANMESVLNKGLALIIGEFGGYHTNGDVDEYAIMKYGQEKGVGWLAWSWYGNNSDLSYLDLATGPNGSLTSFGNTVVNDTYGIKNTSQKAGIY

SEQ ID NO: 22 - protein, 296 aa, Paenibacillus amylolyticus
ATGFYVSGNKLYDSTGKAFVMRGVNHGHSWFKNDLNTAIPAIAKTGANTVRIVLSNGSLYTKDDLNAVKNIINVVNQNKMIAVLEVHDATGKDDYNSLDAAVNYWISIKEALIGKEDRVIVNIANEWYGTWNGSAWADGYKKAIPKLRNAGIKNTLIVDAAGWGQFPQSIVDYGQSVFATDSQKNTVFSIHMYEYAGKDAATVKANMENVLNKGLALIIGEFGGYHTNGDVDEYAIMRYGQEKGVGWLAWSWYGNSSGLNYLDMATGPNGSLTSFGNTVVNDTYGIKKTSQKAGIF

SEQ ID NO: 23 - protein, 297 aa, unknown
  Paenibacillus sp. N021 strain
ASGFYVSGNKLYDSTGKPFVMRGINHGHSWFKNDLNTAIPAIAKTGANTVRIVLSNGTLYTKDDLNSVKNIINLVNQNKMIAVLEVHDATGKDDYNSLDAAVNYWISIKEALIGKEDRVIVNIANEWYGTWNGSAWADGYKKAIPKLRNAGIKNTLIVDAAGWGQYPQSIVDYGQSVFATDTLKNTVFSIHMYEYAGKDAATVKANMENVLNKGLAVIIGEFGGYHTNGDVDEYAIMRYGQEKGVGWLAWSWYGNSSGLGYLDLATGPNGSLTSYGNTVVNDTYGIKNTSQKAGIFQ

SEQ ID NO: 24 - protein, 296 aa, Paenibacillus tundrae
ATGFYVSGGKLYDSTGKAFVMRGVNHGHSWFKNDLNTAIPAIAKTGANTVRIVLSNGVQYTKDDLNSVKNIINVVSVNKMIAVLEVHDATGKDDYNSLDAAVNYWISIKEALIGKEDRVIVNIANEWYGTWNGSAWADGYKKAIPKLRNAGIKNTLIVDAAGWGQYPQSIVDYGQSVFAADSQKNTVFSIHMYEYAGKDAATVKANMESVLNKGLALIIGEFGGYHTNGDVDEYAIMKYGQEKGVGWLAWSWYGNSSDLNYLDLATGPNGSLTSFGNTVVNDTYGIKNTSKKAGIY

SEQ ID NO: 25 - protein, 296 aa, Bacillus circulans CGMCC1554
ATGFYVNGGKLYDSTGKPFYMRGINHGHSWFKNDLNTAIPAIAKTGANTVRIVLSNGTQYTKDDLNSVKNIINVVNANKMIAVLEVHDATGKDDFNSLDAAVNYWISIKEALIGKEDRVIVNIANEWYGTWNGSAWADGYKKAIPKLRDAGIKNTLIVDAAGWGQYPQSIVDYGQSVFAADSQKNTAFSIHMYEYAGKDAATVKSNMENVLNKGLALIIGEFGGYHTNGDVDEYAIMKYGLEKGVGWLAWSWYGNSSGLNYLDLATGPNGSLTSYGNTVVNDTYGIKNTSQKAGIF

SEQ ID NO: 26 - protein, 297 aa, Paenibacillus dauci
AATGFYVSGTKLYDSTGKPFAMRGINHAHTWYKNDLNTAIPAIARTGANTVRIVLSNGMQYTKDDVNSVKNIISLVNQNKMVAVLEVHDATGKDDYNSLDAAVNYWISIKDALIGKEDRVIVNIANEWYGTWNGSAWADGYKQAIPKLRNAGIKNTLIVDAAGWGQYPQSIVDYGQSVFAADSQRNTVFSIHMYEYAGKDAATVKANIDGVLNKGLPVIIGEFGGYHTNGDVDEYAIMRYGQEKGIGWLAWSWYGNSTNLNYLDLATGPNGSLTSFGNTVVNDPSGIKATSQKAGIF

SEQ ID NO: 27 - protein, 296 aa, unknown
  Paenibacillus sp.
ATGFYVSGGKLYDSTGKAFVMRGVNHGHSWFKNDLNTAIPAIAKTGANTVRIVLSNGVQYTKDDLNAVKNIINVISANKMIAVLEVHDATGKDDYNSLDAAVNYWISIKEALIGKEDRVIVNIANEWYGTWNGSAWADGYKKAIPKLRNAGINNTLIVDAAGWGQYPQSIVDYGQSVFAADSQKNTVFSIHMYEYAGKDAATVKANMESVLNKGLALIIGEFGGYHTNGDVDEYAIMKYGQEKGVGWLAWSWYGNNSDLSYLDLAMGPNGSLTSFGNTVVNDTYGIKNTSQKAGIY

SEQ ID NO: 28 - protein, 296 aa, Paenibacillus pabuli
AAGFYVSGNKLYDSTGKAFVMRGVNHSHTWFKNDLNTAIPAIAKTGANTVRIVLSNGTQYTKDDLNAVKNIINLVSQNKMIAVLEVHDATGKDDYNSLDAAVNYWISIKEALIGKEDRVIVNIANEWYGTWNGSAWADGYKKAIPKLRNAGIKNTLIVDAAGWGQYPQSIVDYGQSVFAADAQKNTVFSIHMYEYAGKDAATVKANMENVLNKGLALIIGEFGGYHTNGDVDEYAIMKYGQEKGVGWLAWSWYGNNSDLNYLDLATGPNGTLTSFGNTVVYDTYGIKNTSVKAGIY

SEQ ID NO: 29 - protein, 296 aa, unknown
  Paenibacillus sp.
ATGFYVSGTKLYDSTGKPFAMRGINHAHTWYKNDLNTAIPAIARTGANTVRIVLSNGMQYTKDDVNSVKNIISLVNQNKMVAVLEVHDATGKDDYNSLDAAVNYWISIKDALIGKEDRVIVNIANEWYGTWNGSAWADGYKQAIPKLRNAGIKNTLIVDAAGWGQYPQSIVDYGQSVFAADSQRNTVFSIHMYEYAGKDAATVKANIDGVLNKGLPVIIGEFGGYHTNGDVDEYAIMRYGQEKGIGWLAWSWYGNSTNLNYLDLATGPNGSLTSFGNTVVNDPSGIKATSQKAGIF

SEQ ID NO: 30 - protein, 297 aa, unknown
  Paenibacillus sp. FeL05
ATGFYVSGTKLYDSTGKPFVMRGVNHSHTWFKNDLNAAIPAIAKTGANTVRIVLSNGVQYTRDDVNSVKNIISLVNQNKMIAVLEVHDATGKDDYASLDAAINYWISIKDALIGKEDRVIVNIANEWYGTWNGSAWADGYKQAIPKLRNAGIKNTLIVDAAGWGQYPQSIVDYGQSVFAADSLKNTVFSIHMYEYAGGTDAMVKANMEGVLNKGLPLIIGEFGGQHTNGDVDELAIMRYGQQKGVGWLAWSWYGNNSDLSYLDLATGPNGSLTTFGNTVVNDTNGIKATSKKAGIFQ

SEQ ID NO: 31 - protein, 296 aa, unknown
  Paenibacillus sp. CH3
ATGFYVSGTTLYDSTGKPFVMRGVNHSHTWFKNDLNAAIPAIAKTGANTVRIVLSNGVQYTRDDVNSVKNIISLVNQNKMIAVLEVHDATGKDDYASLDAAVNYWISIKDALIGKEDRVIVNIANEWYGTWNGSAWADGYKQAIPKLRNAGIKNTLIVDAAGWGQCPQSIVDYGQSVFAADSLKNTIFSIHMYEYAGGTDAIVKSNMENVLNKGLPLIIGEFGGQHTNGDVDEHAIMRYGQQKGVGWLAWSWYGNNSELSYLDLATGPAGSLTSIGNTIVNDPYGIKATSKKAGIF

SEQ ID NO: 32 - protein, 297 aa, Paenibacillus wulumuqiensis
AATGFYVSGTKLYDSTGKPFAMRGINHAHTWYKNDLSTAIPAIARTGANTVRIVLSNGTQYTKDDINSVKNIISLVNQNKMIAVLEVHDATGKDDYNSLDAAVNYWISIKDALIGKEDRVIVNIANEWYGTWNGSAWADGYKQAIPKLRNAGIKNTLIVDAAGWGQYPQSIADYGQSVFAADSQRNTVFSIHMYEYAGKDAATVRANIDSVLNKGLPVIIGEFGGYHTNGDVDEYAIMRYSQEKGIGWLAWSWYGNSSNLNYLDMATGPNGSLTSFGNTVVNDPSGIKATSQKAGIF

SEQ ID NO: 33 - protein, 296 aa, Paenibacillus polymyxa E681
ASGFYVSGTKLYDSTGKPFVMRGVNHAHTWYKNDLYTAIPAIAQTGANTVRIVLSNGNQYTKDDINSVKNIISLVSNYKMIAVLEVHDATGKDDYASLDAAVNYWISIKDALIGKEDRVIVNIANEWYGSWNGSGWADGYKQAIPKLRNAGIKNTLIVDCAGWGQYPQSINDFGKSVFAADSLKNTVFSIHMYEFAGKDAQTVRTNIDNVLNQGIPLIIGEFGGYHQGADVDETEIMRYGQSKGVGWLAWSWYGNSSNLSYLDLVTGPNGNLTDWGKTVVNGSNGIKETSKKAGIY

SEQ ID NO: 34 - protein, 296 aa, Paenibacillus polymyxa SC2
ASGFYVSGTNLYDSTGKPFVMRGVNHAHTWYKNDLYTAIPAIAKTGANTVRIVLSNGNQYTKDDINSVKNIISLVSNHKMIAVLEVHDATGKDDYASLDAAVNYWISIKDALIGKEDRVIVNIANEWYGSWNGGGWADGYKQAIPKLRNAGIKNTLIVDCAGWGQYPQSINDFGKSVFAADSLKNTVFSIHMYEFAGKDVQTVRTNIDNVLYQGLPLIIGEFGGYHQGADVDETEIMRYGQSKSVGWLAWSWYGNSSNLNYLDLVTGPNGNLTDWGRTVVEGANGIKETSKKAGIF

SEQ ID NO: 35 - protein, 296 aa, unknown
  Paenibacillus sp.
ASGFYVSGTKLYDSTGNPFVMRGVNHAHTWYKNDLYTAIPAIAKTGANTVRIVLSNGTQYTKDDINSVKNIISLVTSYKMIPVLEVHDATGKDDYASLDAAVNYWISIKDALIGKEDRVIVNIANEWYGSWNGGGWADGYKQAIPKLRNAGIKNTLIVDCAGWGQYPQSINDFGKSVFAADSLKNTVFSIHMYEFAGKDVQTVRTNIDNVLNQGLPLIIGEFGGYHQGADVDETEIMRYGQSKGIGWLAWSWYGNSSNLSYLDLVTGPNGNLTDWGRTVVEGTNGIKETSKKAGIY

SEQ ID NO: 36 - protein, 296 aa, Bacillus circulans 196
ATGFYVNGTKLYDSTGKAFVMRGVNHPHTWYKNDLNAAIPAIAQTGANTVRVVLSNGSQWTKDDLNSVNSIISLVSQHQMIAVLEVHDATGKDEYASLEAAVDYWISIKGALIGKEDRVIVNIANEWYGNWNSSGWADGYKQAIPKLRNAGIKNTLIVDAAGWGQYPQSIVDEGAAVFASDQLKNTVFSIHMYEYAGKDAATVKTNMDDVLNKGLPLIIGEFGGYHQGADVDEIAIMKYGQQKEVGWLAWSWYGNSPELNDLDLAAGPSGNLTGWGNTVVHGTDGIQQTSKKAGIY

SEQ ID NO: 37 - protein, 296 aa, unknown
  Paenibacillus sp.
ATGFYVNGTKLYDSTGKAFVMRGVNHPHTWYKNDLNAAIPAIAQTGANTVRVVLSNGSQWIKDDLNAVNSIISLVSQHQMIAVLEVHDATGKDDDASLEAAVDYWIGIKEALIGKEDRVIVNIANEWYGNWNSSGWAEGYKQAIPKLRNAGIKNTLIVDAAGWGQYPQSIVDEGAAVFASDQLKNTVFSIHMYEYAGKDAATVKTNMDDVLNKGLPLIIGEFGGYHQGADVDEIAIMKYGQQKEVGWLAWSWYGNSPELNDLDLAAGPSGNLTGWGNTVVHGTDGIQQTSKKAGIY

SEQ ID NO: 38 - protein, 298 aa, Paenibacillus mucilaginosus
ATGMYVSGTTVYDANGKPFVMRGINHPHAWYKNDLATAIPAIAATGANSVRIVLSNGSQWSKDSLASIQNIIALCEQYRMIAILEVHDATGSDSYTALDNAVNYWIEMKSALIGKERTVIINIANEWYGTWDASGWANGYKQAIPKLRSAGLDHLLMVDAAGWGQYPASIHTMGKEVLAADPRKNTMFSIHMYEYAGGTADQVRSNIDGVLNQGLAVVVGEFGPKHSNGEVDEATIMSYSQQKGVGWLVWSWYGNSSDLNYLDVATGPSGSLTSWGNTVVNGTNGIKATSALASVFGT

SEQ ID NO: 39 - protein, 298 aa, unknown
  Paenibacillus sp.
VKGFYVSGTKLYDATGSPFVMRGVNHAHTWYKNDLATAIPAIAATGSNTIRIVLSNGSKWSLDSLSDVKNILALCDQYKLTAMLEVHDATGSDNASDLNAAVNYWISIKDALIGKEDRVIVNIANEWFGSWGTASWASAYQSAIPALRAAGIKNTLVVDAAGWGQYPTSIFTSGNAVFNSDPLRNTIFSIHMYEYAGGTAATVKSNIDNALAIGVPVIVGEFGFKHTGGDVDEATIMSYSQEKGVGWLAWSWYGNGGGVEYLDLSNGPSGNLTDWGKTVVNGSYGTLATSVLGKIYTT

SEQ ID NO: 40 - protein, 299 aa, Bacillus circulans K1
ASGFYVSGTKLLDATGQPFVMRGVNHAHTWYKDQLSTAIPAIAKTGANTIRIVLANGHKWTLDDVNTVNNILTLCEQNKLIAVLEVHDATGSDSLSDLDNAVNYWIGIKSALIGKEDRVIINIANEWYGTWDGVAWANGYKQAIPKLRNAGLTHTLIVDSAGWGQYPDSVKNYGTEVLNADPLKNTVFSIHMYEYAGGNASTVKSNIDGVLNKNLALIIGEFGGQHTNGDVDEATIMSYSQEKGVGWLAWSWKGNSSDLAYLDMTNDWAGNSLTSFGNTVVNGSNGIKATSVLSGIFGG

SEQ ID NO: 41 - protein, 299 aa, unknown
  Bacillus sp.
ASGFYVSGTILCDSTGNPFKIRGINHAHSWFKNDSATAMEAIAATGANTVRIVLSNGQQYAKDDANTVSNLLSLANQHKLIAILEVHDATGSDSVSALDHAVDYWIEMKNVLVGKEDRVLINIANEWYGTWDSNGWADGYKSAIPKLRNAGINHTLIVDAAGWGQYPQSIVDKGNEVFNSDPLRNTIFSIHMYEYAGGNADMVRANIDQVLNKGLAVIIGEFGHYHTGGDVDETAIMSYTQQKGVGWLAWSWKGNGAEWLYLDLSYDWAGNHLTEWGETIVNGANGLKATSTRAPIFGN

SEQ ID NO: 42 - protein, 295 aa, Bacillus nealsonii
ASGFYVSGTTLYDATGKPFTMRGVNHAHSWFKEDSAAAIPAIAATGANTVRIVLSDGGQYTKDDINTVKSLLSLAEKINLHSGVMTHRKDDVESLNRAVDYWISLKDTLIGKEDKVIINIANEWYGTWDGAAWAAGYKQAIPKLRNAGLNHTLIIDSAGWGQYPASIHNYGKEVFNADPLKNTMFSIHMYEYAGGDAATVKSNIDGVLNQGLALIIGEFGQKHTNGDVDEATIMSYSQQKNIGWLAWSWKGNSTDWSYLDLSNDWSGNSLTDWGNTVVNGANGLKATSKLSGVFG

SEQ ID NO: 43 - protein, 299 aa, unknown
  Bacillus sp. JAMB602
NSGFYVSGTTLYDANGNPFVMRGINHGHAWYKDQATTAIEGIANTGANTVRIVLSDGGQWTKDDIQTVRNLISLAEDNNLVAVLEVHDATGYDSIASLNRAVDYWIEMRSALIGKEDTVIINIANEWFGSWDGAAWADGYKQAIPRLRNAGLNNTLMIDAAGWGQFPQSIHDYGREVFNADPQRNTMFSIHMYEYAGGNASQVRTNIDRVLNQDLALVIGEFGHRHTNGDVDESTIMSYSEQRGVGWLAWSWKGNGPEWEYLDLSNDWAGNNLTAWGNTIVNGPYGLRETSKLSTVFTG

SEQ ID NO: 44 - protein, 309 aa, unknown
  Bacillus sp..
ANSGFYVSGTTLYDANGNPFVMRGINHGHAWYKDQATTAIEGIANTGANTVRIVLSDGGQWTKDDIHTVRNLISLAEDNHLVAVLEVHDATGYDSIASLNRAVDYWIEMRSALIGKEDTVIINIANEWFGSWEGDAWADGYKQAIPRLRNAGLNHTLMVDAAGWGQFPQSIHDYGREVFNADPQRNTMFSIHMYEYAGGNASQVRTNIDRVLNQDLALVIGEFGHRHTNGDVDEATIMSYSEQRGVGWLAWSWKGNGPEWEYLDLSNDWAGNNLTAWGNTIVNGPYGLRETSRLSTVFTGGGSDGGTSP

SEQ ID NO: 45 - protein, 293 aa, unknown
  Bacillus sp. N165
GFSVDGNTLYDANGQPFVMRGINHGHAWYKDTASTAIPAIAEQGANTIRIVLSDGGQWEKDDIDTIREVIELAEQNKMVAVVEVHDATGRDSRSDLNRAVDYWIEMKDALIGKEDTVIINIANEWYGSWDGSAWADGYIDVIPKLRDAGLTHTLMVDAAGWGQYPQSIHDYGQDVFNADPLKNTMFSIHMYEYAGGDANTVRSNIDRVIDQDLALVIGEFGHRHTDVDEDTILSYSEETGTGWLAWSWKGNSTSWDYLDLSEDWAGQHLTDWGNRIVHGADGLQETSKPSTVF

SEQ ID NO: 46 - protein, 297 aa, artificial sequence
  PspMan variant
MATGFYVSGNKLYDSTGKEFVMRGVNHGHSWFKNDLNEAIPAIAKTGANTVRIVLSNGSLYTLDDLNAVKDIINVVNQNKMIAVLEVHDATGKDDYNSLDAAVNYWISIKEALIGKEDRVIVNIANEWMGTWNGSAWADGYKKAIPKLRNAGIKNTLIVDAAGWGQFPQSIVDYGQSVFAADSLKNTVFSIHMYEYAGKDAATVKANMENVLNKGLALIIGEFGGYHTNGDVDEYAIMRYGQELGVGWLAWSWYGNSDGLRYLDMATGPNGSLTSFGNTVVNDTYGIKNTSQKAGIF

SEQ ID NO: 47 - protein, 297 aa, artificial sequence
  PspMan variant
MATGFYVSGNKLYDSTGKPFVMRGVNHGHSWFKNDLNTAIPAIAKTGANTVRIVLSNGSLYTKDDLDAVKNIINVVNQNKMIAVLEVHDATGKDDYNSLDAAVNYWISIKEALIGKEDRVIVNIANEWMGTWNGSAWADGYKKAIPKLRNAGIKNTLIVDAAGWGQFSQSIVDYGQSVFAADSLKNTVFSIHMYEYAGKDAATVKANMENVLNKGLALIIGEFGGYHTNGDVDEYAIMRYGQELGVGWLAWSWYGNSDPLNYLDMATGPNGSLTSFGNTVVNDTYGIKNTSQKAGIF

SEQ ID NO: 48 - protein, 297 aa, artificial sequence
  PspMan variant
MATGFYVSGNKLYDSTGKEFVMRGVNHGHSWFKNDLNTAIPAIAKTGANTVRIVLSNGSLYTLDDLDAVKNIINVVNDNTMIAVLEVHDATGKDDYDSLDAAVNYWISIKEALIGKEDRVIVNIANEWMGTWNGSAWADGYKKAIPKLRNAGIKNTLIVDAAGWGQFPQSIVDYGQSVFAADSQKNTVFSIHMYEYAGKDAATVKANMENVLNKGLALIIGEFGCYHVNGDVDEYAIMRYGQELGVGWLAWSWYGNSSGLNYLDMATGPNGSLTSFGNTVVNDTYGIKNTSQKAGIF

SEQ ID NO: 49 - protein, 297 aa, artificial sequence
  PspMan variant
MATGFYVSGNKLYDSTGKEFVMRGVNHGHSWFKNDLNEAIPAIAKTGANTVRIVLSNGSLYTKDDLDAVKNIINVVNQNKMIAVLEVHDATGKDDYDSLDAAVNYWISIKEALIGKEDRVIVNIANEWMGTWNGSAWADGYKKAIPKLRNAGIKNTLIVDAAGWGQFSQSIVDYGQSVFAADSLKNTVFSIHMYEYAGKDAATVKANMENVLNKGLALIIGEFGGYHTNGDVDEYAIMRYGQELGVGWLAWSWYGNSDGLRYLDMATGPNGSLTSFGNTVVNDTYGIKNTSQKAGIF

SEQ ID NO: 50 - protein, 297 aa, artificial sequence
  PspMan variant
MATGFYVSGNKLYDSTGKEFVMRGVNHGHSWFKNDLNEAIPAIAKTGANTVRIVLSNGSLYTKDDLDAVKDIINVVNDNTMIAVLEVHDATGKDDYDSLDAAVNYWISIKEALIGKEDRVIVNIANEWMGTWNGSAWADGYKKAIPKLRNAGIKNTLIVDAAGWGQFSQSIVDYGQSVFAADSQKNTVFSIHMYEYAGKDAATVKANMENVLNKGLALIIGEFGCYHTNGDVDEYAIMRYGQELGVGWLAWSWYGNSDGLRYLDMATGPNGSLTSFGNTVVNDTYGIKNTSQKAGIF

SEQ ID NO: 51 - protein, 297 aa, artificial sequence
  PspMan variant
MATGFYVSGNKLYDSTGKPFVMRGVNHGHSWFKNDLNEAIPAIAKTGANTVRIVLSNGSLYTLDDLNAVKDIINVVNQNKMIAVLEVHDATGKDDYDSLDAAVNYWISIKEALIGKEDRVIVNIANEWMGTWNGSAWADGYKKAIPKLRNAGIKNTLIVDAAGWGQFPQSIVDYGQSVFAADSLKNTVFSIHMYEYAGKDAATVKANMENVLNKGLALIIGEFGCYHVNGDVDEYAIMRYGLELGVGWLAWSWYGNSDGLRYLDMATGPNGSLTSFGNTVVNDTYGIKNTSQKAGIF

SEQ ID NO: 52 - protein, 297 aa, artificial sequence
  PspMan variant
MATGFYVSGNKLYDSTGKEFVMRGVNHGHSWFKNDLNTAIPAIAKTGANTVRIVLSNGSLYTLDDLNAVKDIINVVNQNKMIAVLEVHDATGKDDYDSLDAAVNYWISIKEALIGKEDRVIVNIANEWMGTWNGSAWADGYKKAIPKLRNAGIKNTLIVDAAGWGQFPQSIVDYGQSVFAADSLKNTVFSIHMYEYAGKDAATVKANMENVLNKGLALIIGEFGCYHTNGDVDEYAIMRYGQELGVGWLAWSWYGNSDPLNYLDMATGPNGSLTSFGNTVVNDTYGIKNTSQKAGIF

SEQ ID NO: 53 - protein, 298 aa, artificial sequence
  PspMan variant
MATGFYVSGTKLYDSTGKPFVMRGVNHGHSWFKNDLNEAIPAIAKTGANTVRIVLSNGVQYTRDDVNSVKNIISLVNQNKMIAVLEVHDATGKDDYDSLDAAINYWISIKEALIGKEDRVIVNIANEWMGTWNGSAWADGYKKAIPKLRNAGIKNTLIVDAAGWGQYPQSIVDYGQSVFAADSLKNTVFSIHMYEYAGKDAATVKANMENVLNKGLPLIIGEFGCYHTNGDVDELAIMRYGQELGVGWLAWSWYGNSDGLRYLDMATGPNGSLTSFGNTVVNDTYGIKNTSQKAGIFQ

SEQ ID NO: 54 - protein, 297 aa, artificial sequence
  PspMan variant
MATGFYVSGNKLYDSTGKEFVMRGVNHGHSWFKNDLNEAIPAIAKTGANTVRIVLSNGSLYTKDDLDAVKDIINVVNQNKMIAVLEVHDATGKDDYDSLDAAVNYWISIKEALIGKEDRVIVNIANEWMGTWNGSAWADGYKKAIPKLRNAGIKNTLIVDAAGWGQYPQSIVDYGQSVFAADSLKNTVFSIHMYEYAGKDAATVKANMENVLNKGLPLIIGEFGGYHTNGDVDEYAIMRYGQELGVGWLAWSWYGNSDGLRYLDMATGPNGSLTSFGNTVVNDTYGIKNTSQKAGIF

SEQ ID NO: 55 - protein, 297 aa, artificial sequence
  PspMan variant
MATGFYVSGNKLYDSTGKPFVMRGVNHGHSWFKNDLNEAIPAIAKTGANTVRIVLSNGSLYTLDDLDAVKNIINVVNDNTMIAVLEVHDATGKDDYDSLDAAVNYWISIKEALIGKEDRVIVNIANEWMGTWNGSAWADGYKKAIPKLRNAGIKNTLIVDAAGWGQFSQSIVDYGQSVFAADSLKNTVFSIHMYEYAGKDAATVKANMENVLNKGLALIIGEFGGYHTNGDVDEYAIMRYGQELGVGWLAWSWYGNSDGLRYLDMATGPNGSLTSFGNTVVNDTYGIKNTSQKAGIF

SEQ ID NO: 56 - protein, 297 aa, artificial sequence
  PspMan variant
MATGFYVSGNKLYDSTGKEFVMRGVNHGHSWFKNDLNEAIPAIAKTGANTVRIVLSNGSLYTKDDLDAVKNIINVVNQNKMIAVLEVHDATGKDDYNSLDAAVNYWISIKEALIGKEDRVIVNIANEWMGTWNGSAWADGYKKAIPKLRNAGIKNTLIVDAAGWGQFSQSIVDYGQSVFAADSLKNTVFSIHMYEYAGKDAATVKANMENVLNKGLALIIGEFGGYHTNGDVDEYAIMRYGQELGVGWLAWSWYGNSDGLRYLDMATGPNGSLTSFGNTVVNDTYGIKNTSQKAGIF

SEQ ID NO: 57 - protein, 297 aa, artificial sequence
  PspMan variant
MATGFYVSGNKLYDSTGKEFVMRGVNHGHSWFKNDLNTAIPAIAKTGANTVRIVLSNGSLYTKDDLDAVKNIINVVNQNKMIAVLEVHDATGKDDYDSLDAAVNYWISIKEALIGKEDRVIVNIANEWMGTWNGSAWADGYKKAIPKLRNAGIKNTLIVDAAGWGQFSQSIVDYGQSVFAADSLKNTVFSIHMYEYAGKDAATVKANMENVLNKGLALIIGEFGGYHTNGDVDEYAIMRYGQELGVGWLAWSWYGNSSGLNYLDMATGPNGSLTSFGNTVVNDTYGIKNTSQKAGIF

SEQ ID NO: 58 - protein, 297 aa, artificial sequence
  PspMan variant
MATGFYVSGNKLYDSTGKEFVMRGVNHGHSWFKNDLNEAIPAIAKTGANTVRIVLSNGSLYTLDDLNAVKDIINVVNQNKMIAVLEVHDATGKDDYNSLDAAVNYWISIKEALIGKEDRVIVNIANEWMGTWNGSAWADGYKKAIPKLRNAGIKNTLIVDAAGWGQFSQSIVDYGQSVFAADSQKNTVFSIHMYEYAGKDAATVKANMENVLNKGLALIIGEFGCYHVNGDVDEYAIMRYGQELGVGWLAWSWYGNSDGLRYLDMATGPNGSLTSFGNTVVNDTYGIKNTSQKAGIF

SEQ ID NO: 59 - protein, 297 aa, artificial sequence
  PspMan variant
MATGFYVSGNKLYDSTGKEFVMRGVNHGHSWFKNDLNEAIPAIAKTGANTVRIVLSNGSLYTKDDLDAVKNIINVVNQNKMIAVLEVHDATGKDDYDSLDAAVNYWISIKEALIGKEDRVIVNIANEWYGTWNGSAWADGYKKAIPKLRNAGIKNTLIVDAAGWGQFPQSIVDYGQSVFAADSLKNTVFSIHMYEYAGKDAATVKANMENVLNKGLPLIIGEFGCYHVNGDVDELAIMRYGQELGVGWLAWSWYGNSDGLRYLDMATGPNGSLTSFGNTVVNDTYGIKNTSQKAGIF

SEQ ID NO: 60 - protein, 298 aa, artificial sequence
  PspMan variant
MATGFYVSGTKLYDSTGKEFVMRGVNHSHTWFKNDLNEAIPAIAKTGANTVRIVLSNGSLYTKDDLDAVKDIINVVNQNKMIAVLEVHDATGKDDYDSLDAAVNYWISIKEALIGKEDRVIVNIANEWMGTWNGSAWADGYKKAIPKLRNAGIKNTLIVDAAGWGQFSQSIVDYGQSVFAADSLKNTVFSIHMYEYAGKDAATVKANMENVLNKGLALIIGEFGCYHTNGDVDELAIMRYGQELGVGWLAWSWYGNSDGLRYLDMATGPNGSLTSFGNTVVNDTYGIKNTSQKAGIFQ

SEQ ID NO: 61 - protein, 298 aa, artificial sequence
  PspMan variant
MATGFYVSGNKLYDSTGKEFVMRGVNHGHSWFKNDLNEAIPAIAKTGANTVRIVLSNGVQYTRDDLDAVKNIINVVNQNKMIAVLEVHDATGKDDYDSLDAAINYWISIKEALIGKEDRVIVNIANEWMGTWNGSAWADGYKQAIPKLRNAGIKNTLIVDAAGWGQYPQSIVDYGQSVFAADSLKNTVFSIHMYEYAGKDAATVKANMENVLNKGLALIIGEFGCYHTNGDVDELAIMRYGQELGVGWLAWSWYGNSDGLRYLDMATGPNGSLTSFGNTVVNDTYGIKNTSQKAGIFQ

SEQ ID NO: 62 - protein, 298 aa, artificial sequence
  PspMan variant
MATGFYVSGNKLYDSTGKEFVMRGVNHGHSWFKNDLNEAIPAIAKTGANTVRIVLSNGSLYTKDDLDAVKDIINVVNDNTMIAVLEVHDATGKDDYDSLDAAVNYWISIKEALIGKEDRVIVNIANEWMGTWNGSAWADGYKKAIPKLRNAGIKNTLIVDAAGWGQFSQSIVDYGQSVFAADSQKNTVFSIHMYEYAGKDAATVKANMENVLNKGLALIIGEFGCYHVNGDVDEYAIMRYGQELGVGWLAWSWYGNSDGLRYLDMATGPNGSLTSFGNTVVNDTYGIKNTSQKAGIFQ

SEQ ID NO: 63 - protein, 298 aa, artificial sequence
  PspMan variant
MATGFYVSGNKLYDSTGKEFVMRGVNHGHSWFKNDLNEAIPAIAKTGANTVRIVLSNGVQYTLDDLNAVRDIINVVNDNTMIAVLEVHDATGKDDYDSLDAAVNYWISIKDALIGKEDRVIVNIANEWMGTWNGSAWADGYKKAIPKLRNAGIKNTLIVDAAGWGQFPQSIVDYGQSVFAADSLKNTVFSIHMYEYAGKDAATVKANMENVLNKGLALIIGEFGCYHVNGDVDELAIMRYGQELGVGWLAWSWYGNSDGLRYLDMATGPNGSLTSFGNTVVNDTYGIKNTSQKAGIFQ

SEQ ID NO: 64 - protein, 298 aa, artificial sequence
  PspMan variant
MATGFYVSGTKLYDSTGKPFVMRGVNHGHSWFKNDLNEAIPAIAKTGANTVRIVLSNGSLYTLDDLNAVKDIINVVNQNKMIAVLEVHDATGKDDYDSLDAAINYWISIKEALIGKEDRVIVNIANEWMGTWNGSAWADGYKKAIPKLRNAGIKNTLIVDAAGWGQYPQSIVDYGQSVFAADSLKNTVFSIHMYEYAGKDAATVKANMENVLNKGLALIIGEFGCYHVNGDVDELAIMRYGQELGVGWLAWSWYGNSDGLRYLDMATGPNGSLTSFGNTVVNDTYGIKNTSQKAGIFQ

SEQ ID NO: 65 - protein, 298 aa, artificial sequence
  PspMan variant
MATGFYVSGTKLYDSTGKEFVMRGVNHGHSWFKNDLNEAIPAIAKTGANTVRIVLSNGSLYTKDDLDAVKNIINVVNDNTMIAVLEVHDATGKDDYDSLDAAVNYWISIKEALIGKEDRVIVNIANEWMGTWNGSAWADGYKQAIPKLRNAGIKNTLIVDAAGWGQFPQSIVDYGQSVFAADSLKNTVFSIHMYEYAGKDAATVKANMENVLNKGLPLIIGEFGCYHVNGDVDELAIMRYGQELGVGWLAWSWYGNSDGLRYLDMATGPNGSLTSFGNTVVNDTYGIKNTSQKAGIFQ

SEQ ID NO: 66 - protein, 298 aa, artificial sequence
  PspMan variant
MATGFYVSGTKLYDSTGKEFVMRGVNHGHSWFKNDLNEAIPAIAKTGANTVRIVLSNGVQYTLDDLNAVKNIINVVNQNKMIAVLEVHDATGKDDYDSLDAAINYWISIKEALIGKEDRVIVNIANEWMGTWNGSAWADGYKKAIPKLRNAGIKNTLIVDAAGWGQYPQSIVDYGQSVFAADSLKNTVFSIHMYEYAGKDAATVKANMENVLNKGLALIIGEFGCYHTNGDVDELAIMRYGQELGVGWLAWSWYGNSDGLRYLDMATGPNGSLTSFGNTVVNDTYGIKNTSQKAGIFQ

SEQ ID NO: 67 - protein, 298 aa, artificial sequence
  PspMan variant
MATGFYVSGNKLYDSTGKEFVMRGVNHGHTWFKNDLNEAIPAIAKTGANTVRIVLSNGVQYTRDDLDAVKNIINVVNDNTMIAVLEVHDATGKDDYDSLDAAVNYWISIKEALIGKEDRVIVNVANEWMGTWNGSAWADGYKQAIPKLRNAGIKNTLIVDAAGWGQYPQSIVDYGQSVFAADSLKNTVFSIHMYEYAGKDAATVKANMENVLNKGLALIIGEFGCYHTNGDVDELAIMRYGQELGVGWLAWSWYGNSDGLRYLDMATGPNGSLTSFGNTVVNDTYGIKNTSQKAGIFQ

SEQ ID NO: 68 - protein, 298 aa, artificial sequence
  PspMan variant
MATGFYVSGSKLYDSTGKEFVMRGVNHGHTWFKNDLNEAIPAIAKTGANTVRIVLSNGVQYTLDDLDAVKNIINVVNHNTMMAVLEVHDATGKDDYDSLDAAVNYWISIKEALIGKEDRVIVNIANEWMGTWNGSAWADGYKQAIPKLRNAGIKNTLIVDAAGWGQYPQSIVDYGQSVFAADSLKNTVFSIHMYEYAGKDAATVKANMENVLNKGLALIIGEFGCYHTNGDVDELAIMRYGQELGVGWLAWSWYGNSDGLRYLDMATGPNGSLTSFGNTVVNDTYGIKNTSQKAGIFQ

SEQ ID NO: 69 - protein, 298 aa, artificial sequence
  PspMan variant
MATGFYVSGTKLYDSTGKEFVMRGVNHGHTWFKNDLNEAIPAIAKTGANTVRIVLSNGVQYTRDDLDAVKNIINVVNQNKMIAVLEVHDATGKDDYDSLDAAVNYWISIKEALIGKEDRVIVNIANEWMGTWNGSAWADGYKQAIPKLRNAGIKNTLIVDAAGWGQFSQSIVDYGQSVFAADSLKNTVFSIHMYEYAGKDAATVKANMENVLNKGLALIIGEFGCYHVNGDVDELAIMRYGQELGVGWLAWSWYGNSDGLRYLDMATGPNGSLTSFGNTVVNDTYGIKNTSQKAGIFQ

SEQ ID NO: 70 - protein, 298 aa, artificial sequence
  PspMan variant
MATSFYVSGTKLYDSTGKEFVMRGVNHGHSWFKNDLNEAIPAIAKTGANTVRIVLSNGSLYTKDDLDAVKNIINVVNDNTMIAVLEVHDATGKDDYDSLDAAVNYWISIKEALIGKEDRVIVNIANEWMGTWNGSAWADGYKKAIPKLRNAGIKNTLIVDAAGWGQFPQSIVDYGQSVFAADSLKNTVFSIHMYEYAGKDAATVKANMENVLNKGLALIIGEFGCYHVNGDVDELAIMRYGQELGVGWLAWSWYGNSDGLRYLDMATGPNGSLTSFGNTVVNDTYGIKNTSQKAGIFQ

SEQ ID NO: 71 - protein, 298 aa, artificial sequence
  PspMan variant
MATGFYVSGTKLYDSTGKEFVMRGVNHGHTWFKNDLNEAIPAIAKTGANTVRIVLSNGVQYTLDDLNAVRDIINVVNDNTMIAVLEVHDATGKDDYDSLDAAVNYWISIKEALIGKEDRVIVNIANEWMGAWNGSAWADGYKKAIPKLRNAGIKNTLIVDAAGWGQYPQSIVDYGQSVFAADSLKNTVFSIHMYEYAGKDAATVKANMENVLNKGLALIIGEFGCYHTNGDVDELAIMRYGQELGVGWLAWSWYGNSDGLRYLDMATGPNGSLTSFGNTVVNDTYGIKNTSQKAGIFQ

SEQ ID NO: 72 - protein, 298 aa, artificial sequence
  PspMan variant
MATGFYVSGTKLYDSTGKEFVMRGVNHGHTWFKNDLNEAIPAIAKTGANTVRIVLSNGVQYTLDDLNAVRDIINVVNDNTMIAVLEVHDATGKDDYDSLDAAVNYWISIKDALIGKEDRVIVNIANEWMGTWNGSAWADGYKKAIPKLRNAGIKNTLIVDAAGWGQFSQSIVDYGQSVFAADSLKNTVFSIHMYEYAGKDAATVKANMENVLNKGLALIIGEFGCYHVNGDVDELAIMRYGQELGVGWLAWSWYGNSDGLRYLDMATGPNGSLTSFGNTVVNDTYGIKNTSQKAGIFQ

SEQ ID NO: 73 - protein, 298 aa, artificial sequence
  PspMan variant
MATGFYVSGNKLYDSTGKEFVMRGVNHGHTWFKNDLNEAIPAIAKTGANTVRIVLSNGVQYTRDDLDAVKNIINVVNQNKMIAVLEVHDATGKDDYDSLDAAVNYWISIKEALIGKEDRVIVNIANEWMGTWNGSAWADGYKKAIPKLRNAGIKNTLIVDAAGWGQFSQSIVDYGQSVFAADSLKNTVFSIHMYEYAGKDAATVKANMENVLNIGLALIIGEFGCYHTNGDVDELAIMRYGQELGVGWLAWSWYGNSDGLRYLDMATGPNGSLTSFGNTVVNDTYGIKNTSQKAGIFQ

SEQ ID NO: 74 - protein, 298 aa, artificial sequence
  PspMan variant
MATGFYVSGTKLYDSTGKEFVMRGVNHGHTWFKNDLNEAIPAIAKTGANTVRIVLSNGVQYTRDDLDAVKNIINVVNQNKMIAVLEVHDATGKDDYDSLDAAVNYWISIKEALIGKEDRVIVNIANEWMGTWNGSAWADGYKQAIPKLRNAGIKNTLIVDAAGWGQFSQSIVDYGQSVFAADSLKNTVFSIHMYEYAGKDAATVKANMENVLNKGLALIIGEFGPYHVNGDVDELAIMRYGQELGVGWLAWSWYGNSDGLRYLDMATGPNGSLTSFGNTVVNDTYGIKNTSQKAGIFQ

SEQ ID NO: 75 - protein, 298 aa, artificial sequence
  PspMan variant
VATGFYVSGNKLYDSTGKEFVMRGVNHGHTWFKNDLNEAIPAIAKTGANTVRIVLSNGSLYEKDDLDAVKDIINVVNDNKMIAVLEVHDATGKDDYDSLDAAVNYWISIKEALIGKEDRVIVNIANEWMGTWNGSAWADGYKRAIPKLRNAGIKNTLIVDAAGWGQYSQSIVDYGQSVFAADSLKNTVFSIHMYEYAGKDAATVKANMENVLNKGLALIIGEFGCYHTNGDVDELAIMRYGQELGVGWLAWSWYGNSDGLRYLDMATGPNGSLTSFGNTVVNDAYGIKNTSQKAGIFQ

SEQ ID NO: 76 - protein, 298 aa, artificial sequence
  PspMan variant
MATGFEVSGTKLYDSTGKEFVMRGVNHSHTWFKNDLNEAIPAIAKTGANTVRIVLSNGSLYTLDDLDAVKDIINVVNQNKMIAVLEVHDATGKDDYDSLDAAVNYWISIKSALIGKEDRVIVNIANEWMGTWNGLAWADGYKKAIPKLRNAGIKNTLIVDAAGWGQFSQSIVDYGQSVFAADSLKNTVFSIHMYEYAGKDAATVKANMENVLNKGLALIIGEFGCYHVNGDVDELAIMRYGQELGVGWLAWSWYGNSDGLQYLDMATGPNGSLTSFGNTVVNSTYGIKNTSQKAGIFQ

SEQ ID NO: 77 - protein, 298 aa, artificial sequence
  PspMan variant
MATGFYVSGTKLYDSTGKEFVMRGVNHGHTWFKNDLNEAIPAIAKTGANTVRIVLSNGVQYTRDDLDAVKDIINVVNQNKMIAVLEVHDATGKDDYDSLDAAINYWISIKEALIGKEDRVIVNIANEWMGTWNGSAWADGYKQAIPKLRNAGIKNTLIVDAAGWGQFSQSIVDYGQSVFAADSLKNTVFSIHMYEYAGKDAATVKANMENVLNKGLALIIGEFGPYHVNGDVDELAIMRYGQELGVGWLAWSWYGNSDGLRYLDMATGPNGSLTSFGNTVVNDTYGIKNTSQKAGIFQ

SEQ ID NO: 78 - protein, 298 aa, artificial sequence
  PspMan variant
MSTGFYVSGNKLYDSTGKEFVMRGVNHSHTWFKNDLNEAIPAIAKTGANTVRIVLSNGSLYTRDDLDAVKDIIEVVNQNKMIAVLEVHDATGRDDYDSLDAAVNYWISIKEALIGKEDRVIVNIANEWMGTWNGSAWADGYKKAIPKLRTAGIKNTLIVDAAGWGQFSQSIVDYGQSVFAADSLKNTVFSIHMYEYAGKDAATVKANMENVLAKGLALIIGEFGCYHTNGDVDELAIMRYGQELGVGWLAWSWYGNSDGLQYLDMATGPNGSLTSFGNTVVNDTYGIKNTSQKAGIFQ

SEQ ID NO: 79 - protein, 298 aa, artificial sequence
  PspMan variant
LATGFYVSGTKLYDSTGKEFVMRGVNHAHTWFKNDLNEAIPAIAKTGANTVRIVLSNGSLYTLDDLDAVKDIINVVNDNKMIAVLEVHDATGKDDYDSLDAAVNYWISIKEALIGKEDRVIVNIANEWMGTWNGSLWADGYKKAIPKLRNAGIKNTLIVDAAGWGQFAQSIVDYGQSVFAADSLKNTVFSIHMYEYAGKDAATVKANMENVLAKGLALIIGEFGCYHTNGDVDELAIMRYGQELGVGWLAWSWYGNSDGLRYLDMATGPNGSLTSFGNTVVNDTYGIKNTSQKAGIFQ

SEQ ID NO: 80 - protein, 298 aa, artificial sequence
  PspMan variant
MATGFYVSGNKLYDSTGKEFVMRGVNHGHSWFKNDLNEAIPAIAKTGANTVRIVLSNGVLYTRDDLDAVKNIINVVNQNKMIAVLEVHDATGKDDYDSLDAAINYWISIKEALIGKEDRVIVNIANEWMGTWNGSAWADGYKKAIPKLRNAGIKNTLIVDAAGWGQYPQSIVDYGQSVFAADSLKNTVFSIHMYEYAGKDAATVKANMENVLNKGLALIIGEFGCYHVNGDVDELAIMRYGQELGVGWLAWSWYGNSDGLRYLDMATGPNGSLTSFGNTVVNDTYGIKNTSQKAGIFQ

SEQ ID NO: 81 - protein, 298 aa, artificial sequence
  PspMan variant
MATGFYVSGTKLYDSTGKEFVMRGVNHAHTWFKNDLNEAIPAIAKTGANTVRIVLSNGSLYTRDDLDAVKNIINVVNQNKMIAVLEVHDATGKDDYDSLDAAVNYWISIKEALIGKEDRVIVNIANEWMGTWNGSAWADGYKKAIPKLRNAGIKNTLIVDAAGWGQFPQSIVDYGQSVFAADSLKNTVFSIHMYEYAGKDAATVKANMENVLNKGLALIIGEFGCYHVNGDVDELAIMRYGQELGVGWLAWSWYGNSDGLRYLDMATGPNGSLTSFGNTVVNDTYGIKNTSQKAGIFQ

SEQ ID NO: 82 - protein, 298 aa, artificial sequence
  PspMan variant
MARGFYVSGTKLYDSTGKEFVMRGVNHAHTWFKNDLNEAIPAIAKTGANTVRIVLSNGSLYEKDDLDAVKDIINVVNQNKMIAVLEVHDATGRDDYLSLDAAVNYWISIKSALIGKEDRVIVNIANEWMGTWNGSAWAMGYKKAIPKLRNAGIKNTLIVDAAGWGQFSQSIVDYGQSVFAADSLKNTVFSIHMYEYAGKDAATVKANMENVLNKGLALIIGEFGCYHTNGDVDELAIMRYGQELGVGWLAWSWYGNSDGLQYLDMATGPNGSLTSFGNTVVNDTYGIKNTSQKAGIFQ

SEQ ID NO: 83 - protein, 298 aa, artificial sequence
  PspMan variant
MATGFYVSGTKLYDSTGKEFVMRGVNHAHTWFKNDLNEAIPAIAKTGANTVRIVLSNGDLYTKDDLDSVKDIINVVNQNKMIAVLEVHDATGRDDYDSLDAAVNYWISIKEALIGKEDRVIVNIANEWMGTWNGSAWADGYKQAIPKLRNAGIKNTLIVDAAGWGQFSQSIVDYGQSVFAADSDKNTVFSIHMYEYAGKDAATVKANMENVLNKGLALIIGEFGCYHTNGDVDELAIMRYGQELGVGWLAWSWYGNSDGLRYLDMATGPNGSLTSFGNTVVNDEYGIKNTSQKAGIFQ

SEQ ID NO: 84 - protein, 297 aa, artificial sequence
  PspMan variant
MATGFYVSGNKLYDSTGKEFVMRGVNHGHSWFKNDLNTAIPAIAKTGANTVRIVLSNGSLYTLDDLNAVKDIINVVNQNKMIAVLEVHDATGKDDYNSLDAAVNYWISIKEALIGKEDRVIVNIANEWMGTWNGSAWADGYKKAIPKLRNAGIKNTLIVDAAGWGQFSQSIVDYGQSVFAADSLKNTVFSIHMYEYAGKDAATVKANMENVLNKGLALIIGEFGCYHTNGDVDEYAIMRYGQELGVGWLAWSWYGNSSRLNYLDMATGPNGSLTSFGNTVVNDTYGIKNTSQKAGIF

SEQ ID NO: 85 - protein, 297 aa, artificial sequence
  PspMan variant
MATGFYVSGNKLYDSTGKEFVMRGVNHGHSWFKNDLNTAIPAIAKTGANTVRIVLSNGSLYTKDDLDAVKDIINVVNDNTMIAVLEVHDATGKDDYDSLDAAVNYWISIKEALIGKEDRVIVNIANEWMGTWNGSAWADGYKKAIPKLRNAGIKNTLIVDAAGWGQFSQSIVDYGQSVFAADSLKNTVFSIHMYEYAGKDAATVKANMENVLNKGLALIIGEFGGYHTNGDVDEYAIMRYGQELGVGWLAWSWYGNSSGLNYLDMATGPNGSLTSFGNTVVNDTYGIKNTSQKAGIF

SEQ ID NO: 86 - protein, 297 aa, artificial sequence
  PspMan variant
MATGFYVSGNKLYDSTGKEFVMRGVNHGHSWFKNDLNEAIPAIAKTGANTVRIVLSNGSLYTKDDLDAVKNIINVVNQNKMIAVLEVHDATGKDDYNSLDAAVNYWISIKEALIGKEDRVIVNIANEWMGTWNGSAWADGYKKAIPKLRNAGIKNTLIVDAAGWGQFSQSIVDYGQSVFAADSLKNTVFSIHMYEYAGKDAATVKANMENVLNKGLALIIGEFGGYHVNGDVDEYAIMRYGQELGVGWLAWSWYGNSSGLNYLDMATGPNGSLTSFGNTVVNDTYGIKNTSQKAGIF

SEQ ID NO: 87 - protein, 297 aa, artificial sequence
  PspMan variant
MATGFYVSGNKLYDSTGKEFVMRGVNHGHSWFKNDLNEAIPAIAKTGANTVRIVLSNGSLYTKDDLDAVKNIINVVNQNKMIAVLEVHDATGKDDYNSLDAAVNYWISIKEALIGKEDRVIVNIANEWMGTWNGSAWADGYKKAIPKLRNAGIKNTLIVDAAGWGQFPQSIVDYGQSVFAADSLKNTVFSIHMYEYAGKDAATVKANMENVLNKGLALIIGEFGGYHTNGDVDEYAIMRYGQELGVGWLAWSWYGNSDGLRYLDMATGPNGSLTSFGNTVVNDTYGIKNTSQKAGIF

SEQ ID NO: 88 - protein, 297 aa, artificial sequence
  PspMan variant
MATGFYVSGNKLYDSTGKEFVMRGVNHGHSWFKNDLNTAIPAIAKTGANTVRIVLSNGSLYTLDDLNAVKDIINVVNQNKMIAVLEVHDATGKDDYNSLDAAVNYWISIKEALIGKEDRVIVNIANEWMGTWNGSAWADGYKKAIPKLRNAGIKNTLIVDAAGWGQFSQSIVDYGQSVFAADSLKNTVFSIHMYEYAGKDAATVKANMENVLNKGLALIIGEFGGYHTNGDVDEYAIMRYGQELGVGWLAWSWYGNSDGLRYLDMATGPNGSLTSFGNTVVNDTYGIKNTSQKAGIF

SEQ ID NO: 89 - protein, 297 aa, artificial sequence
  PspMan variant
MATGFYVSGNKLYDSTGKEFVMRGVNHGHSWFKNDLNEAIPAIAKTGANTVRIVLSNGSLYTLDDLNAVKDIINVVNQNKMIAVLEVHDATGKDDYNSLDAAVNYWISIKEALIGKEDRVIVNIANEWMGTWNGSAWADGYKKAIPKLRNAGIKNTLIVDAAGWGQFSQSIVDYGQSVFAADSLKNTVFSIHMYEYAGKDAATVKANMENVLNKGLALIIGEFGGYHTNGDVDEYAIMRYGQELGVGWLAWSWYGNSDPLNYLDMATGPNGSLTSFGNTVVNDTYGIKNTSQKAGIF

SEQ ID NO: 90 - protein, 297 aa, artificial sequence
  PspMan variant
MATGFYVSGNKLYDSTGKPFVMRGVNHGHSWFKNDLNTAIPAIAKTGANTVRIVLSNGSLYTLDDLNAVKDIINVVNQNKMIAVLEVHDATGKDDYNSLDAAVNYWISIKEALIGKEDRVIVNIANEWMGTWNGSAWADGYKRAIPKLRNAGIKNTLIVDAAGWGQFSQSIVDYGQSVFAADSLKNTVFSIHMYEYAGKDAATVKANMENVLNKGLALIIGEFGCYHVNGDVDEYAIMRYGQELGVGWLAWSWYGNSDPLNYLDMATGPNGSLTSFGNTVVNDTYGIKNTSQKAGIF

SEQ ID NO: 91 - protein, 297 aa, artificial sequence
  PspMan variant
MATGFYVSGNKLYDSTGKEFVMRGVNHGHSWFKNDLNEAIPAIAKTGANTVRIVLSNGSLYTLDDLNAVKDIINVVNQNKMIAVLEVHDATGKDDYNSLDAAVNYWISIKEALIGKEDRVIVNIANEWMGTWNGSAWADGYKKAIPKLRNAGIKNTLIVDAAGWGQFSQSIVDYGQSVFAADSLKNTVFSIHMYEYAGKDAATVKANMENVLNKGLALIIGEFGGYHTNGDVDEYAIMRYGQELGVGWLAWSWYGNSDGLRYLDMATGPNGSLTSFGNTVVNDTYGIKNTSQKAGIF

SEQ ID NO: 92 - DNA, 87 bp, unknown
  Paenibacillus sp.
gtgagaagcaaaaaattgtggatcagcttgttgtttgcgttaacgttaatctttacgatggcgttcagcaacatgtctgcgcaggct

SEQ ID NO: 93 - DNA, 894 bp, artificial sequence
  nucleic acid sequence coding for PSpMan variant
atggcgacaggcttttatgtttcaggcaacaaactgtatgatagcacaggcaaagagtttgttatgaggggcgttaatcatggccatagctggtttaaaaacgatctgaatgaggcgattccggctattgcaaaaacaggcgcaaatacagttagaattgttctgtcaaatggcagcctgtatacgctggatgatctgaatgcagtcaaagacatcatcaatgtcgtcaaccagaacaaaatgattgcagttctggaagttcatgatgcaacgggcaaagatgattacaattcactggatgcagcagtcaactattggatctcaattaaagaagcgctgatcggcaaagaagatcgcgttattgttaatattgcgaacgaatggatgggcacatggaatggctcagcatgggcagatggctacaaaaaagcaattccgaaactgagaaatgcaggcatcaaaaacacactgattgttgatgcggcaggctggggacaatttccgcaatcaattgttgactatggccaaagcgtttttgcagcagatagcttgaaaaatacagtctttagcatccatatgtacgaatacgctggaaaagatgcagcaacagttaaagcgaatatggaaaacgtcctgaataaaggcctggcactgattattggcgaatttggcggatatcatacaaatggcgacgttgatgaatatgcgattatgagatatggccaagaactgggcgttggctggcttgcatggtcatggtatggaaattcagacggccttcggtatctggatatggcaacaggaccgaatggatcactgacatcatttggcaatacagtcgtcaatgatacgtatggaatcaaaaatacgagccagaaagctgggatcttttaa

SEQ ID NO: 94 - DNA, 894 bp, artificial sequence
  nucleic acid sequence coding for PSpMan variant
atggcgacaggcttttatgtttcaggcaacaaactgtatgatagcacaggcaaaccgtttgttatgagaggcgttaatcatggccatagctggtttaaaaacgatctgaatacagcgattccggctattgcaaaaacaggcgcaaatacagttagaattgttctgtcaaatggcagcctgtatacgaaagatgatctggacgcagtcaaaaacatcatcaatgtcgtcaaccagaacaaaatgattgcagttctggaagttcatgatgcaacgggcaaagatgattacaattcactggatgcagcagtcaactattggatctcaattaaagaagcgctgatcggcaaagaagatcgcgttattgttaatattgcgaacgaatggatgggcacatggaatggctcagcatgggcagatggctacaaaaaagcaattccgaaactgagaaatgcaggcatcaaaaacacactgattgttgatgcggcaggctggggacaattttcccaatcaattgttgattatggccaaagcgtttttgcagcagatagcttgaaaaatacagtctttagcatccatatgtacgaatacgctggaaaagatgcagcaacagttaaagcgaatatggaaaacgtcctgaataaaggcctggcactgattattggcgaatttggcggatatcatacaaatggcgacgttgatgaatatgcgattatgagatatggccaagaattgggcgttggctggcttgcatggtcatggtatggaaattcagacccccttaactatctggatatggcaacaggaccgaatggatcactgacatcatttggcaatacagtcgtcaatgatacgtatggaatcaaaaatacgagccagaaagctggcatcttttaa

SEQ ID NO: 95 - DNA, 894 bp, artificial sequence
  nucleic acid sequence coding for PSpMan variant
atggcgacaggcttttatgtttcaggcaacaaactgtatgatagcacaggcaaagagtttgttatgagaggcgttaatcatggccatagctggtttaaaaacgatctgaatacagcgattccggctattgcaaaaacaggcgcaaatacagttagaattgttctgtcaaatggcagcctgtatacgctggatgatctggacgcagtcaaaaacatcatcaatgtcgtcaacgacaacacgatgattgcagttctggaagttcatgatgcaacgggcaaagatgattacgattcactggatgcagcagtcaactattggatctcaattaaagaagcgctgatcggcaaagaagatcgcgttattgttaatattgcgaacgaatggatgggcacatggaatggctcagcatgggcagatggctacaaaaaagcaattccgaaactgagaaatgcaggcatcaaaaacacactgattgttgatgcggcaggctggggacaatttccgcaatcaattgttgattatggccaaagcgtttttgcagcagatagccagaaaaatacagtctttagcatccatatgtacgaatacgctggaaaagatgcagcaacagttaaagcgaatatggaaaacgtcctgaataaaggcctggcactgattattggcgaatttggctgctatcatgtgaatggcgacgttgatgaatatgcgattatgagatatggccaagaactgggcgttggctggcttgcatggtcatggtatggaaattcatcaggccttaactatctggatatggcaacaggaccgaatggatcactgacatcatttggcaatacagtcgtcaatgatacgtatggaatcaaaaatacgagccagaaagctggcatcttttaa

SEQ ID NO: 96 - DNA, 894 bp, artificial sequence
  nucleic acid sequence coding for PSpMan variant
atggcgacaggcttttatgtttcaggcaacaaactgtatgatagcacaggcaaagagtttgttatgagaggcgttaatcatggccatagctggtttaaaaacgatctgaatgaggcgattccggctattgcaaaaacaggcgcaaatacagttagaattgttctgtcaaatggcagcctgtatacgaaagatgatctggacgcagtcaaaaacatcatcaatgtcgtcaaccagaacaaaatgattgcagttctggaagttcatgatgcaacgggcaaagatgattacgattcactggatgcagcagtcaactattggatctcaattaaagaagcgctgatcggcaaagaagatcgcgttattgttaatattgcgaacgaatggatgggcacatggaatggctcagcatgggcagatggctacaaaaaagcaattccgaaactgagaaatgcaggcatcaaaaacacactgattgttgatgcggcaggctggggacaattttcccaatcaattgttgattatggccaaagcgtttttgcagcagatagcttgaaaaatacagtctttagcatccatatgtacgaatacgctggaaaagatgcagcaacagttaaagcgaatatggaaaacgtcctgaataaaggcctggcactgattattggcgaatttggcggatatcatacaaatggcgacgttgatgaatatgcgattatgagatatggccaagaattgggcgttggctggcttgcatggtcatggtatggaaattcagacggccttcggtatctggatatggcaacaggaccgaatggatcactgacatcatttggcaatacagtcgtcaatgatacgtatggaatcaaaaatacgagccagaaagctggcatcttttaa

SEQ ID NO: 97 - DNA, 894 bp, artificial sequence
  nucleic acid sequence coding for PSpMan variant
atggcgacaggcttttatgtttcaggcaacaaactgtatgatagcacaggcaaagagtttgttatgagaggcgttaatcatggccatagctggtttaaaaacgatctgaatgaggcgattccggctattgcaaaaacaggcgcaaatacagttagaattgttctgtcaaatggcagcctgtatacgaaagatgatctggacgcagtcaaagacatcatcaatgtcgtcaacgacaacacgatgattgcagttctggaagttcatgatgcaacgggcaaagatgattacgattcactggatgcagcagtcaactattggatctcaattaaagaagcgctgatcggcaaagaagatcgcgttattgttaatattgcgaacgaatggatgggcacatggaatggctcagcatgggcagatggctacaaaaaagcaattccgaaactgagaaatgcaggcatcaaaaacacactgattgttgatgcggcaggctggggacaattttcccaatcaattgttgattatggccaaagcgtttttgcagcagatagccagaaaaatacagtctttagcatccatatgtacgaatacgctggaaaagatgcagcaacagttaaagcgaatatggaaaacgtcctgaataaaggcctggcactgattattggcgaatttggctgctatcatacaaatggcgacgttgatgaatatgcgattatgagatatggccaagaattgggcgttggctggcttgcatggtcatggtatggaaattcagacggccttcggtatctggatatggcaacaggaccgaatggatcactgacatcatttggcaatacagtcgtcaatgatacgtatggaatcaaaaatacgagccagaaagctggcatcttttaa

SEQ ID NO: 98 - DNA, 894 bp, artificial sequence
  nucleic acid sequence coding for PSpMan variant
atggcgacaggcttttatgtttcaggcaacaaactgtatgatagcacaggcaaaccgtttgttatgagaggcgttaatcatggccatagctggtttaaaaacgatctgaatgaggcgattccggctattgcaaaaacaggcgcaaatacagttagaattgttctgtcaaatggcagcctgtatacgctggatgatctgaatgcagtcaaagacatcatcaatgtcgtcaaccagaacaaaatgattgcagttctggaagttcatgatgcaacgggcaaagatgattacgattcactggatgcagcagtcaactattggatctcaattaaagaagcgctgatcggcaaagaagatcgcgttattgttaatattgcgaacgaatggatgggcacatggaatggctcagcatgggcagatggctacaaaaaagcaattccgaaactgagaaatgcaggcatcaaaaacacactgattgttgatgcggcaggctggggacaatttccgcaatcaattgttgactatggccaaagcgtttttgcagcagatagcttgaaaaatacagtctttagcatccatatgtacgaatacgctggaaaagatgcagcaacagttaaagcgaatatggaaaacgtcctgaataaaggcctggcactgattattggcgaatttggctgctatcatgtgaatggcgacgttgatgaatatgcgattatgagatatggcctagaattgggcgttggctggcttgcatggtcatggtatggaaattcagacggccttcggtatctggatatggcaacaggaccgaatggatcactgacatcatttggcaatacagtcgtcaatgatacgtatggaatcaaaaatacgagccagaaagctggcatcttttaa

SEQ ID NO: 99 - DNA, 894 bp, artificial sequence
  nucleic acid sequence coding for PSpMan variant
atggcgacaggcttttatgtttcaggcaacaaactgtatgatagcacaggcaaagagtttgttatgagaggcgttaatcatggccatagctggtttaaaaacgatctgaatacagcgattccggctattgcaaaaacaggcgcaaatacagttagaattgttctgtcaaatggcagcctgtatacgctggatgatctgaatgcagtcaaagacatcatcaatgtcgtcaaccagaacaaaatgattgcagttctggaagttcatgatgcaacgggcaaagatgattacgattcactggatgcagcagtcaactattggatctcaattaaagaagcgctgatcggcaaagaagatcgcgttattgttaatattgcgaacgaatggatgggcacatggaatggctcagcatgggcagatggctacaaaaaagcaattccgaaactgagaaatgcaggcatcaaaaacacactgattgttgatgcggcaggctggggacaatttccgcaatcaattgttgactatggccaaagcgtttttgcagcagatagcttgaaaaatacagtctttagcatccatatgtacgaatacgctggaaaagatgcagcaacagttaaagcgaatatggaaaacgtcctgaataaaggcctggcactgattattggcgaatttggctgctatcatacaaatggcgacgttgatgaatatgcgattatgagatatggccaagaattgggcgttggctggcttgcatggtcatggtatggaaattcagacccccttaactatctggatatggcaacaggaccgaatggatcactgacatcatttggcaatacagtcgtcaatgatacgtatggaatcaaaaatacgagccagaaagctggcatcttttaa

SEQ ID NO: 100 - DNA, 897 bp, artificial sequence
  nucleic acid sequence coding for PSpMan variant
atggcgacaggcttttatgtttcaggcaccaaactgtatgatagcacaggcaaaccgtttgttatgagaggcgttaatcatggccatagctggtttaaaaacgatctgaatgaggcgattccggctattgcaaaaacaggcgcaaatacagttagaattgttctgtcaaatggcgtgcagtatacgagagatgatgtaaattccgtcaaaaacatcatctctctcgtcaaccagaacaaaatgattgcagttctggaagttcatgatgcaacgggcaaagatgattacgattcactggatgcagcaatcaactattggatctcaattaaagaagcgctgatcggcaaagaagatcgcgttattgttaatattgcgaacgaatggatgggcacatggaatggctcagcatgggcagatggctacaaaaaagcaattccgaaactgagaaatgcaggcatcaaaaacacactgattgttgatgcggcaggctggggacaatatccgcaatcaattgttgattatggccaaagcgtttttgcagcagatagcttaaaaaatacagtctttagcatccatatgtacgaatacgctggaaaagatgcagcaacagttaaagcgaatatggaaaacgtcctgaataaaggcctgccactgattattggcgaatttggctgctatcatacaaatggcgacgttgatgaactggcgattatgagatatggccaagaattgggcgttggctggcttgcatggtcatggtatggaaattcagacggccttcggtatctggatatggcaacaggaccgaatggatcactgacatcatttggcaatacagtcgtcaatgatacgtatggaatcaaaaatacgagccagaaagctggcatctttcagtaa

SEQ ID NO: 101 - DNA, 894 bp, artificial sequence
  nucleic acid sequence coding for PSpMan variant
atggcgacaggcttttatgtttcaggcaacaaactgtatgatagcacaggcaaagagtttgttatgagaggcgttaatcatggccatagctggtttaaaaacgatctgaatgaggcgattccggctattgcaaaaacaggcgcaaatacagttagaattgttctgtcaaatggcagcctgtatacgaaagatgatctggacgcagtcaaagacatcatcaatgtcgtcaaccagaacaaaatgattgcagttctggaagttcatgatgcaacgggcaaagatgattacgattcactggatgcagcagtcaactattggatctcaattaaagaagcgctgatcggcaaagaagatcgcgttattgttaatattgcgaacgaatggatgggcacatggaatggctcagcatgggcagatggctacaaaaaagcaattccgaaactgagaaatgcaggcatcaaaaacacactgattgttgatgcggcaggctggggacaatatccgcaatcaattgttgactatggccaaagcgtttttgcagcagatagcttgaaaaatacagtctttagcatccatatgtacgaatacgctggaaaagatgcagcaacagttaaagcgaatatggaaaacgtcctgaataaaggcctgccactgattattggcgaatttggcggatatcatacaaatggcgacgttgatgaatatgcgattatgagatatggccaagaattgggcgttggctggcttgcatggtcatggtatggaaattcagacggccttcggtatctggatatggcaacaggaccgaatggatcactgacatcatttggcaatacagtcgtcaatgatacgtatggaatcaaaaatacgagccagaaagctggcatcttttaa

SEQ ID NO: 102 - DNA, 894 bp, artificial sequence
  nucleic acid sequence coding for PSpMan variant
atggcgacaggcttttatgtttcaggcaacaaactgtatgatagcacaggcaaaccgtttgttatgagaggcgttaatcatggccatagctggtttaaaaacgatctgaatgaggcgattccggctattgcaaaaacaggcgcaaatacagttagaattgttctgtcaaatggcagcctgtatacgctggatgatctggacgcagtcaaaaacatcatcaatgtcgtcaacgacaacacgatgattgcagttctggaagttcatgatgcaacgggcaaagatgattacgattcactggatgcagcagtcaactattggatctcaattaaagaagcgctgatcggcaaagaagatcgcgttattgttaatattgcgaacgaatggatgggcacatggaatggctcagcatgggcagatggctacaaaaaagcaattccgaaactgagaaatgcaggcatcaaaaacacactgattgttgatgcggcaggctggggacaattttcccaatcaattgttgattatggccaaagcgtttttgcagcagatagcttgaaaaatacagtctttagcatccatatgtacgaatacgctggaaaagatgcagcaacagttaaagcgaatatggaaaacgtcctgaataagggcctggcactgattattggcgaatttggcggatatcatacaaatggcgacgttgatgaatatgcgattatgagatatggccaagaattgggcgttggctggcttgcatggtcatggtatggaaattcagacggccttcggtatctggatatggcaacaggaccgaatggatcactgacatcatttggcaatacagtcgtcaatgatacgtatggaatcaaaaatacgagccagaaagctggcatcttttaa

SEQ ID NO: 103 - DNA, 894 bp, artificial sequence
  nucleic acid sequence coding for PSpMan variant
atggcgacaggcttttatgtttcaggcaacaaactgtatgatagcacaggcaaagagtttgttatgagaggcgttaatcatggccatagctggtttaaaaacgatctgaatgaggcgattccggctattgcaaaaacaggcgcaaatacagttagaattgttctgtcaaatggcagcctgtatacgaaagatgatctggacgcagtcaaaaacatcatcaatgtcgtcaaccagaacaaaatgattgcagttctggaagttcatgatgcaacgggcaaagatgattacaattcactggatgcagcagtcaactattggatctcaattaaagaagcgctgatcggcaaagaagatcgcgttattgttaatattgcgaacgaatggatgggcacatggaatggctcagcatgggcagatggctacaaaaaagcaattccgaaactgagaaatgcaggcatcaaaaacacactgattgttgatgcggcaggctggggacaattttcccaatcaattgttgattatggccaaagcgtttttgcagcagatagcttgaaaaatacagtctttagcatccatatgtacgaatacgctggaaaagatgcagcaacagttaaagcgaatatggaaaacgtcctgaataaaggcctggcactgattattggcgaatttggcggatatcatacaaatggcgacgttgatgaatatgcgattatgagatatggccaagaattgggcgttggctggcttgcatggtcatggtatggaaattcagacggccttcggtatctggatatggcaacaggaccgaatggatcactgacatcatttggcaatacagtcgtcaatgatacgtatggaatcaaaaatacgagccagaaagctggcatcttttaa

SEQ ID NO: 104 - DNA, 894 bp, artificial sequence
  nucleic acid sequence coding for PSpMan variant
atggcgacaggcttttatgtttcaggcaacaaactgtatgatagcacaggcaaagagtttgttatgaggggcgttaatcatggccatagctggtttaaaaacgatctgaatacagcgattccggctattgcaaaaacaggcgcaaatacagttagaattgttctgtcaaatggcagcctgtatacgaaagatgatctggacgcagtcaaaaacatcatcaatgtcgtcaaccagaacaaaatgattgcagttctggaagttcatgatgcaacgggcaaagatgattacgattcactggatgcagcagtcaactattggatctcaattaaagaagcgctgatcggcaaagaagatcgcgttattgttaatattgcgaacgaatggatgggcacatggaatggctcagcatgggcagatggctacaaaaaagcaattccgaaactgagaaatgcaggcatcaaaaacacactgattgttgatgcggcaggctggggacaattttcccaatcaattgttgattatggccaaagcgtttttgcagcagatagcttgaaaaatacagtctttagcatccatatgtacgaatacgctggaaaagatgcagcaacagttaaagcgaatatggaaaacgtcctgaataaaggcctggcactgattattggcgaatttggcggatatcatacaaatggcgacgttgatgaatatgcgattatgagatatggccaagaactgggcgttggctggcttgcatggtcatggtatggaaattcatcaggccttaactatctggatatggcaacaggaccgaatggatcactgacatcatttggcaatacagtcgtcaatgatacgtatggaatcaaaaatacgagccagaaagctggcatcttttaa

SEQ ID NO: 105 - DNA, 894 bp, artificial sequence
  nucleic acid sequence coding for PSpMan variant
atggcgacaggcttttatgtttcaggcaacaaactgtatgacagcacaggcaaagagtttgttatgagaggcgttaatcatggccatagctggtttaaaaacgatctgaatgaggcgattccggctattgcaaaaacaggcgcaaatacagttagaattgttctgtcaaatggcagcctgtatacgctggatgatctgaatgcagtcaaagacatcatcaatgtcgtcaaccagaacaaaatgattgcagttctggaagttcatgatgcaacgggcaaagatgattacaattcactggatgcagcagtcaactattggatctcaattaaagaagcgctgatcggcaaagaagatcgcgttattgttaatattgcgaacgaatggatgggcacatggaatggctcagcatgggcagatggctacaaaaaagcaattccgaaactgagaaatgcaggcatcaaaaacacactgattgttgatgcggcaggctggggacaattttcccaatcaattgttgattatggccaaagcgtttttgcagcagatagccagaaaaatacagtctttagcatccatatgtacgaatacgctggaaaagatgcagcaacagttaaagcgaatatggaaaacgtcctgaataaaggcctggcactgattattggcgaatttggctgctatcatgtgaatggcgacgttgatgaatatgcgattatgagatatggccaagaattgggcgttggctggctcgcatggtcatggtatggaaattcagacggccttcggtatctggatatggcaacaggaccgaatggatcactgacatcatttggcaatacagtcgtcaatgatacgtatggaatcaaaaatacgagccagaaagctggcatcttttaa

SEQ ID NO: 106 - DNA, 894 bp, artificial sequence
  nucleic acid sequence coding for PSpMan variant
atggcgacaggcttttatgtttcaggcaacaaactgtatgatagcacaggcaaagagtttgttatgagaggcgttaatcatggccatagctggtttaaaaacgatctgaatgaggcgattccggctattgcaaaaacaggcgcaaatacagttagaattgttctgtcaaatggcagcctgtatacgaaagatgatctggacgcagtcaaaaacatcatcaatgtcgtcaaccagaacaaaatgattgcagttctggaagttcatgatgcaacgggcaaagatgattacgattcactggatgcagcagtcaactattggatctcaattaaagaagcgctgatcggcaaagaagatcgcgttattgttaatattgcgaacgaatggtatggcacatggaatggctcagcatgggcagatggctacaaaaaagcaattccgaaactgagaaatgcaggcatcaaaaacacactgattgttgatgcggcaggctggggacaatttccgcaatcaattgttgattatggccaaagcgtttttgcagcagatagcttaaaaaatacagtctttagcatccatatgtacgaatacgctggaaaagatgcagcaacagttaaagcgaatatggaaaacgtcctgaataaaggcctgccactgattattggcgaatttggctgctatcatgtgaatggcgacgttgatgaactggcgattatgagatatggccaagaattgggcgttggctggcttgcatggtcatggtatggaaattcagacggccttcggtatctggatatggcaacaggaccgaatggatcactgacatcatttggcaatacagtcgtcaatgatacgtatggaatcaaaaatacgagccagaaagctggcatcttttaa

SEQ ID NO: 107 - DNA, 897 bp, artificial sequence
  nucleic acid sequence coding for PSpMan variant
atggcgacaggcttttatgtttcaggcaccaaactgtatgatagcacaggcaaagagtttgttatgagaggcgttaatcattcccatacctggtttaaaaacgatctgaatgaggcgattccggctattgcaaaaacaggcgcaaatacagttagaattgttctgtcaaatggcagcctgtatacgaaagatgatctggacgcagtcaaagacatcatcaatgtcgtcaaccagaacaaaatgatagcagttctggaagttcatgatgcaacgggcaaagatgattacgattcactggatgcagcagtcaactattggatctcaattaaagaagcgctgatcggcaaagaagatcgcgttattgttaatattgcgaacgaatggatgggcacatggaatggctcagcatgggcagatggctacaaaaaagcaattccgaaactgagaaatgcaggcatcaaaaacacactgattgttgatgcggcaggctggggacaattttcccaatcaattgttgattatggccaaagcgtttttgcagcagatagcttgaaaaatacagtctttagcatccatatgtacgaatacgctggaaaagatgcagcaacagttaaagcgaatatggaaaacgtcctgaataaaggcctggcactgattattggcgaatttggctgctatcatacaaatggcgacgttgatgaactggcgattatgagatatggccaagaattgggcgttggctggcttgcatggtcatggtatggaaattcagacggccttcggtatctggatatggcaacaggaccgaatggatcactgacatcatttggcaatacagtcgtcaatgatacgtatggaatcaaaaatacgagccagaaagctggcatctttcagtaa

SEQ ID NO: 108 - DNA, 897 bp, artificial sequence
  nucleic acid sequence coding for PSpMan variant
atggcgacaggcttttatgtttcaggcaacaaactgtatgatagcacaggcaaagagtttgttatgagaggcgttaatcatggccatagctggtttaaaaacgatctgaatgaggcgattccggctattgcaaaaacaggcgcaaatacagttagaattgttctgtcaaatggcgtgcagtatacgagagatgatctggacgcagtcaaaaacatcatcaatgtcgtcaaccagaacaaaatgattgcagttctggaagttcatgatgcaacgggcaaagatgattacgattcactggatgcagcaatcaactattggatctcaattaaagaagcgctgatcggcaaagaagatcgcgttattgttaatattgcgaacgaatggatgggcacatggaatggctcagcatgggcagatggctacaaacaggcaattccgaaactgagaaatgcaggcatcaaaaacacactgattgttgatgcggcaggctggggacaatatccgcaatcaattgttgattatggccaaagcgtttttgcagcagatagcttaaaaaatacagtctttagcatccatatgtacgaatacgctggaaaagatgcagcaacagttaaagcgaatatggaaaacgtcctgaataaaggcctggcactgattattggcgaatttggctgctatcatacaaatggcgacgttgatgaactggcgattatgagatatggccaagaattgggcgttggctggcttgcatggtcatggtatggaaattcagacggccttcggtatctggatatggcaacaggaccgaatggatcactgacatcatttggcaatacagtcgtcaatgatacgtatggaatcaaaaatacgagccagaaagctggcatctttcagtaa

SEQ ID NO: 109 - DNA, 897 bp, artificial sequence
  nucleic acid sequence coding for PSpMan variant
atggcgacaggcttttatgtttcaggcaacaaactgtatgacagcacaggcaaagagtttgttatgagaggcgttaatcatggccatagctggtttaaaaacgatctgaatgaggcgattccggctattgcaaaaacaggcgcaaatacagttagaattgttctgtcaaatggcagcctgtatacgaaagatgatctggacgcagtcaaagacatcatcaatgtcgtcaacgacaacacgatgattgcagttctggaagttcatgatgcaacgggcaaagatgattacgattcactggatgcagcagtcaactattggatctcaattaaagaagcgctgatcggcaaagaagatcgcgttattgttaatattgcgaacgaatggatgggcacatggaatggctcagcatgggcagatggctacaaaaaagcaattccgaaactgagaaatgcaggcatcaaaaacacactgattgttgatgcggcaggctggggacaattttcccaatcaattgttgactatggccaaagcgtttttgcagcagatagccagaaaaatacagtctttagcatccatatgtacgaatacgctggaaaagatgcagcaacagttaaagcgaatatggaaaacgtcctgaataaaggcctggcactgattattggcgaatttggctgctatcatgtgaatggcgacgttgatgaatatgcgattatgagatatggccaagaattgggcgttggctggcttgcatggtcatggtatggaaattcagacggccttcggtatctggatatggcaacaggaccgaatggatcactgacatcatttgggaatacagtcgtcaatgatacgtatggaatcaaaaatacgagccagaaagctggcatctttcagtaa

SEQ ID NO: 110 - DNA, 897 bp, artificial sequence
  nucleic acid sequence coding for PSpMan variant
atggcgacaggcttttatgtttcaggcaacaaactgtatgatagcacaggcaaagagtttgttatgagaggcgttaatcatggccatagctggtttaaaaacgatctgaatgaggcgattccggctattgcaaaaacaggcgcaaatacagttagaattgttctgtcaaatggcgtgcagtatacgctggatgatctgaatgcagtcagagacatcatcaatgtcgtcaacgacaacacgatgattgcagttctggaagttcatgatgcaacgggcaaagatgattacgattcactggatgcagcagtcaactattggatctcaattaaagatgcgctgatcggcaaagaagatcgcgttattgttaatattgcgaacgaatggatgggcacatggaatggctcagcatgggcagatggctacaaaaaagcaattccgaaactgagaaatgcaggcatcaaaaacacactgattgttgatgcggcaggctggggacaatttccgcaatcaattgttgactatggccaaagcgtttttgcagcagatagcttaaaaaatacagtctttagcatccatatgtacgaatacgctggaaaagatgcagcaacagttaaagcgaatatggaaaacgtcctgaataaaggcctggcactgattattggcgaatttggctgctatcatgtgaatggcgacgttgatgaactggcgattatgagatatggccaagaattgggcgttggctggcttgcatggtcatggtatggaaattcagacggccttcggtatctggatatggcaacaggaccgaatggatcactgacatcatttggcaatacagtcgtcaatgatacgtatggaatcaaaaatacgagccagaaagctggcatctttcagtaa

SEQ ID NO: 111 - DNA, 897 bp, artificial sequence
  nucleic acid sequence coding for PSpMan variant
atggcgacaggcttttatgtttcaggcaccaaactgtatgatagcacaggcaaaccgtttgttatgagaggcgttaatcatggccatagctggtttaaaaacgatctgaatgaggcgattccggctattgcaaaaacaggcgcaaatacagttagaattgttctgtcaaatggcagcctgtatacgctggatgatctgaatgcagtcaaagacatcatcaatgtcgtcaaccagaacaaaatgattgcagttctggaagttcatgatgcaacgggcaaagatgattacgattcactggatgcagcaatcaactattggatctcaattaaagaagcgctgatcggcaaagaagatcgcgttattgttaatattgcgaacgaatggatgggcacatggaatggctcagcatgggcagatggctacaaaaaagcaattccgaaactgagaaatgcaggcatcaaaaacacactgattgttgatgcggcaggctggggacaatatccgcaatcaattgttgattatggccaaagcgtttttgcagcagatagcttaaaaaatacagtctttagcatccatatgtacgaatacgctggaaaagatgcagcaacagttaaagcgaatatggaaaacgtcctgaataaaggcctggcactgattattggcgaatttggctgctatcatgtgaatggcgacgttgatgaactggcgattatgagatatggccaagaattgggcgttggctggcttgcatggtcatggtatggaaattcagacggccttcggtatctggatatggcaacaggaccgaatggatcactgacatcatttggcaatacagtcgtcaatgatacgtatggaatcaaaaatacgagccagaaagctggcatctttcagtaa

SEQ ID NO: 112 - DNA, 897 bp, artificial sequence
  nucleic acid sequence coding for PSpMan variant
atggcgacaggcttttatgtttcaggcaccaaactgtatgatagcacaggcaaagagtttgttatgagaggcgttaatcatggccatagctggtttaaaaacgatctgaatgaggcgattccggctattgcaaaaacaggcgcaaatacagttagaattgttctgtcaaatggcagcctgtatacgaaagatgatctggacgcagtcaaaaacatcatcaatgtcgtcaacgacaacacgatgattgcagttctggaagttcatgatgcaacgggcaaagatgattacgattcactggatgcagcagtcaactattggatctcaattaaagaagcgctgatcggcaaagaagatcgcgttattgttaatattgcgaacgaatggatgggcacatggaatggctcagcatgggcagatggctacaaacaggcaattccgaaactgagaaatgcaggcatcaaaaacacactgattgttgatgcggcaggctggggacaatttccgcaatcaattgttgattatggccaaagcgtttttgcagcagatagcttaaaaaatacagtctttagcatccatatgtacgaatacgctggaaaagatgcagcaacagttaaagcgaatatggaaaacgtcctgaataaaggcctgccactgattattggcgaatttggctgctatcatgtgaatggcgacgttgatgaactggcgattatgagatatggccaagaattgggcgttggctggcttgcatggtcatggtatggaaattcagacggccttcggtatctggatatggcaacaggaccgaatggatcactgacatcatttggcaatacagtcgtcaatgatacgtatggaatcaaaaatacgagccagaaagctggcatctttcagtaa

SEQ ID NO: 113 - DNA, 897 bp, artificial sequence
  nucleic acid sequence coding for PSpMan variant
atggcgacaggcttttatgtttcaggcaccaaactgtatgatagcacaggcaaagagtttgttatgagaggcgttaatcatggccatagctggtttaaaaacgatctgaatgaggcgattccggctattgcaaaaacaggcgcaaatacagttagaattgttctgtcaaatggcgtgcagtatacgctggatgatctgaatgcagtcaaaaacatcatcaatgtcgtcaaccagaacaaaatgattgcagttctggaagttcatgatgcaacgggcaaagatgattacgattcactggatgcagcaatcaactattggatctcaattaaagaagcgctgatcggcaaagaagatcgcgttattgttaatattgcgaacgaatggatgggcacatggaatggctcagcatgggcagatggctacaaaaaagcaattccgaaactgagaaatgcaggcatcaaaaacacactgattgttgatgcggcaggctggggacaatatccgcaatcaattgttgattatggccaaagcgtttttgcagcagatagcttgaaaaatacagtctttagcatccatatgtacgaatacgctggaaaagatgcagcaacagttaaagcgaatatggaaaacgtcctgaataaaggcctggcactgattattggcgaatttggctgctatcatacaaatggcgacgttgatgaactggcgattatgagatatggccaagaattgggcgttggctggcttgcatggtcatggtatggaaattcagacggccttcggtatctggatatggcaacaggaccgaatggatcactgacatcatttggcaatacagtcgtcaatgatacgtatggaatcaaaaatacgagccagaaagctggcatctttcagtaa

SEQ ID NO: 114 - DNA, 897 bp, artificial sequence
  nucleic acid sequence coding for PSpMan variant
atggcgacaggcttttatgtttcaggcaacaaactgtatgatagcacaggcaaagagtttgttatgagaggcgttaatcatggccatacctggtttaaaaacgatctgaatgaggcgattccggctattgcaaaaacaggcgcaaatacagttagaattgttctgtcaaatggcgtgcagtatacgagagatgatctggacgcagtcaaaaacatcatcaatgtcgtcaaccagaacaaaatgatagcagttctggaagttcatgatgcaacgggcaaagatgattacgattcactggatgcagcaatcaactattggatctcaattaaagaagcgctgatcggcaaagaagatcgcgttattgttaatattgcgaacgaatggatgggcacatggaatggctcagcatgggcagatggctacaaaaaagcaattccgaaactgagaaatgcaggcatcaaaaacacactgattgttgatgcggcaggctggggacaatatccgcaatcaattgttgattatggccaaagcgtttttgcagcagatagcttaaaaaatacagtctttagcatccatatgtacgaatacgctggaaaggatgcagcaacagttaaagcgaatatggaaaacgtcctgaataaaggcctggcactgattattggcgaatttggctgctatcatgtgaatggcgacgttgatgaactggcgattatgagatatggccaagaattgggcgttggctggcttgcatggtcatggtatggaaattcagacggccttcggtatctggatatggcaacaggaccgaatggatcactgacatcatttggcaatacagtcgtcaatgatacgtatggaatcaaaaatacgagccagaaagctggcatctttcagtaa

SEQ ID NO: 115 - DNA, 897 bp, artificial sequence
  nucleic acid sequence coding for PSpMan variant
atggcgacaggcttttatgtttcaggcaacaaactgtatgatagcacaggcaaagagtttgttatgagaggcgttaatcatggccatacctggtttaaaaacgatctgaatgaggcgattccggctattgcaaaaacaggcgcaaatacagttagaattgttctgtcaaatggcgtgcagtatacgagagatgatctggacgcagtcaaaaacatcatcaatgtcgtcaacgacaacacgatgattgcagttctggaagttcatgatgcaacgggcaaagatgattacgattcactggatgcagcagtcaactattggatctcaattaaagaagcgctgatcggcaaagaagatcgcgttattgttaatgttgcgaacgaatggatgggcacatggaatggctcagcatgggcagatggctacaaacaggcaattccgaaactgagaaatgcaggcatcaaaaacacactgattgttgatgcggcaggctggggacaatatccgcaatcaattgttgattatggccaaagcgtttttgcagcagatagcttaaaaaatacagtctttagcatccatatgtacgaatacgctggaaaagatgcagcaacagttaaagcgaatatggaaaacgtcctgaataaaggcctggcactgattattggcgaatttggctgctatcatacaaatggcgacgttgatgaactggcgattatgagatatggccaagaattgggcgttggctggcttgcatggtcatggtatggaaattcagacggccttcggtatctggatatggcaacaggaccgaatggatcactgacatcatttggcaatacagtcgtcaatgatacgtatggaatcaaaaatacgagccagaaagctggcatctttcagtaa

SEQ ID NO: 116 - DNA, 897 bp, artificial sequence
  nucleic acid sequence coding for PSpMan variant
atggcgacaggcttttatgtttcaggcagcaaactgtatgatagcacaggcaaagagtttgttatgagaggcgttaatcatggccatacctggtttaaaaacgatctgaatgaggcgattccggctattgcaaaaacaggcgcaaatacagttagaattgttctgtcaaatggcgtgcagtatacgctagatgatctggacgcagtcaaaaacatcatcaatgtcgtcaaccacaacacaatgatggcagttctggaagttcatgatgcaacgggcaaagatgattacgattcactggatgcagcagtcaactattggatctcaattaaagaagcgctgatcggcaaagaagatcgcgttattgttaatattgcgaacgaatggatgggcacatggaatggctcagcatgggcagatggctacaaacaagcaattccgaaactgagaaatgcaggcatcaaaaacacactgattgttgatgcggcaggctggggacaatatccgcaatcaattgttgactatggccaaagcgtttttgcagcagatagcttaaaaaatacagtctttagcatccatatgtacgaatacgctggaaaagatgcagcaacagttaaagcgaatatggaaaacgtcctgaataaaggcctggcactgattattggcgaatttggctgctatcatacaaatggcgacgttgatgaactggcgattatgagatatggccaagaattgggcgttggctggcttgcatggtcatggtatggaaattcagacggccttcggtatctggatatggcaacaggaccgaatggatcactgacatcatttggcaatacagtcgtcaatgatacgtatggaatcaaaaatacgagccagaaagctggcatctttcagtaa

SEQ ID NO: 117 - DNA, 897 bp, artificial sequence
  nucleic acid sequence coding for PSpMan variant
atggcgacaggcttttatgtttcaggcaccaaactgtatgatagcacaggcaaagagtttgttatgagaggcgttaatcatggccatacctggtttaaaaacgatctgaatgaggcgattccggctattgcaaaaacaggcgcaaatacagttagaattgttctgtcaaatggcgtgcagtatacgagagatgatctggacgcagtcaaaaacatcatcaatgtcgtcaaccagaacaaaatgattgcagttctggaagttcatgatgcaacgggcaaagatgattacgattcactggatgcagcagtcaactattggatctcaattaaagaagcgctgatcggcaaagaagatcgcgttattgttaatattgcgaacgaatggatgggcacatggaatggctcagcatgggcagatggctacaaacaggcaattccgaaactgagaaatgcaggcatcaaaaacacactgattgttgatgcggcaggctggggacaattttcccaatcaattgttgattatggccaaagcgtttttgcagcagatagcttaaaaaatacagtctttagcatccatatgtacgaatacgctggaaaagatgcagcaacagttaaagcgaatatggaaaacgtcctgaataaaggcctggcactgattattggcgaatttggctgctatcatgtgaatggcgacgttgatgaactggcgattatgagatatggccaagaattgggcgttggctggcttgcatggtcatggtatggaaattcagacggccttcggtatctggatatggcaacaggaccgaatggatcactgacatcatttggcaatacagtcgtcaatgatacgtatggaatcaaaaatacgagccagaaagctggcatctttcagtaa

SEQ ID NO: 118 - DNA, 897 bp, artificial sequence
  nucleic acid sequence coding for PSpMan variant
atggcgacaagcttctatgtttccggcaccaaactgtatgatagcacaggcaaagagtttgttatgagaggcgttaatcatggccatagctggtttaaaaacgatctgaatgaggcgattccggctattgcaaaaacaggcgcaaatacagttagaattgttctgtcaaatggcagcctgtatacgaaagatgatctggacgcagtcaaaaacatcatcaatgtcgtcaacgacaacacgatgattgcagttctggaagttcatgatgcaacgggcaaagatgattacgattcactggatgcagcagtcaactattggatctcaattaaagaagcgctgatcggcaaagaagatcgcgttattgttaatattgcgaacgaatggatgggcacatggaatggctcagcatgggcagatggctacaaaaaagcaattccgaaactgagaaatgcaggcatcaaaaacacactgattgttgatgcggcaggctggggacaatttccgcaatcaattgttgactatggccaaagcgtttttgcagcagatagcttaaaaaatacagtctttagcatccatatgtacgaatacgctggaaaagatgcagcaacagttaaagcgaatatggaaaacgtcctgaataaaggcctggcactgattattggcgaatttggctgctatcatgtgaatggcgacgttgatgaactggcgattatgagatatggccaagaattgggcgttggctggcttgcatggtcatggtatggaaattcagacggccttcggtatctggatatggcaacaggaccgaatggatcactgacatcatttggcaatacagtcgtcaatgatacgtatggaatcaaaaatacgagccagaaagctggcatctttcagtaa

SEQ ID NO: 119 - DNA, 897 bp, artificial sequence
  nucleic acid sequence coding for PSpMan variant
atggcgacaggcttttatgtttcaggcaccaaactgtatgatagcacaggcaaagagtttgttatgagaggcgttaatcatggccatacctggtttaaaaacgatctgaatgaggcgattccggctattgcaaaaacaggcgcaaatacagttagaattgttctgtcaaatggcgtgcagtatacgctggatgatctgaatgcagtcagagacatcatcaatgtcgtcaacgacaacacgatgattgcagttctggaagttcatgatgcaacgggcaaagatgattacgattcactggatgcagcagtcaactattggatctcaattaaagaagcgctgatcggcaaagaagatcgcgttattgttaatattgcgaacgaatggatgggcgcatggaatggctcagcatgggcagatggctacaaaaaagcaattccgaaactgagaaatgcaggcatcaaaaacacactgattgttgatgcggcaggctggggacaatatccgcaatcaattgttgactatggccaaagcgtttttgcagcagatagcttgaaaaatacagtctttagcatccatatgtacgaatacgctggaaaagatgcagcaacagttaaagcgaatatggaaaacgtcctgaataaaggcctggcactgattattggcgaatttggctgctatcatacaaatggcgacgttgatgaactggcgattatgagatatggccaagaattgggcgttggctggcttgcatggtcatggtatggaaattcagacggccttcggtatctggatatggcaacaggaccgaatggatcactgacatcatttggcaatacagtcgtcaatgatacgtatggaatcaaaaatacgagccagaaagctggcatctttcagtaa

SEQ ID NO: 120 - DNA, 897 bp, artificial sequence
  nucleic acid sequence coding for PSpMan variant
atggcgacaggcttttatgtttcaggcaccaaactgtatgatagcacaggcaaagagtttgttatgagaggcgttaatcatggccatacctggtttaaaaacgatctgaatgaggcgattccggctattgcaaaaacaggcgcaaatacagttagaattgttctgtcaaatggcgtgcagtatacgctggatgatctgaatgcagtcagagacatcatcaatgtcgtcaacgacaacacgatgattgcagttctggaagttcatgatgcaacgggcaaagatgattacgattcactggatgcagcagtcaactattggatctcaattaaagatgcgctgatcggcaaagaagatcgtgttattgttaatattgcgaacgaatggatgggcacatggaatggctcagcatgggcagatggctacaaaaaagcaattccgaaactgagaaatgcaggcatcaaaaacacactgattgttgatgcggcaggctggggacaattttcccaatcaattgttgattatggccaaagcgtttttgcagcagatagcttgaaaaatacagtctttagcatccatatgtacgaatacgctggaaaagatgcagcaacagttaaagcgaatatggaaaacgtcctgaataaaggcctggcactgattattggcgaatttggctgctatcatgtgaatggcgacgttgatgaactggcgattatgagatatggccaagaattgggcgttggctggcttgcatggtcatggtatggaaattcagacggccttcggtatctggatatggcaacaggaccgaatggatcactgacatcatttggcaatacagtcgtcaatgatacgtatggaatcaaaaatacgagccagaaagctggcatctttcagtaa

SEQ ID NO: 121 - DNA, 897 bp, artificial sequence
  nucleic acid sequence coding for PSpMan variant
atggcgacaggcttttatgtttcaggcaacaaactgtacgatagcacaggcaaagagtttgttatgagaggcgttaatcatggccatacctggtttaaaaacgatctgaatgaggcgattccggctattgcaaaaacaggcgcaaatacagttagaattgttctgtcaaatggcgtgcagtatacgagagatgatctggacgcagtcaaaaacatcatcaatgtcgtcaaccagaacaaaatgattgcagttctggaagttcatgatgcaacgggcaaagatgattacgattcactggatgcagcagtcaactattggatctcaattaaagaagcgctgatcggcaaagaagatcgcgttattgttaatattgcgaacgaatggatgggcacatggaatggctcagcatgggcagatggctacaaaaaagcaattccgaaactgagaaatgcaggcatcaaaaacacactgattgttgatgcggcaggctggggacaattttcgcaatcaattgttgactatggccaaagcgtttttgcagcagatagcttgaaaaatacagtctttagcatccatatgtacgaatacgctggaaaagacgcagcaacagttaaagcgaatatggaaaacgtcctgaatataggcctggcactgattattggcgaatttggctgctatcatacaaatggcgacgttgatgaactggcgattatgagatatggccaagaattgggcgttggctggcttgcatggtcatggtatggaaattcagacggccttcggtatctggatatggcaacaggaccgaatggatcactgacatcatttggcaatacagtcgtcaatgatacgtatggaatcaaaaatacgagccagaaagctggcatctttcagtaa

SEQ ID NO: 122 - DNA, 897 bp, artificial sequence
  nucleic acid sequence coding for PSpMan variant
atggcgacaggcttttatgtttcaggcaccaaactgtatgatagcacaggcaaagagtttgttatgagaggcgttaatcatggccatacctggtttaaaaacgatctgaatgaggcgattccggctattgcaaaaacaggcgcaaatacagttagaattgttctgtcaaatggcgtgcagtatacgagagatgatctggacgcagtcaaaaacatcatcaatgtcgtcaaccagaacaaaatgattgcagttctggaagttcatgatgcaacgggcaaagatgattacgattcactggatgcagcagtcaactattggatctcaattaaagaagcgctgatcggcaaagaagatcgcgttattgttaatattgcgaacgaatggatgggcacatggaatggctcagcatgggcagatggctacaaacaggcaattccgaaactgagaaatgcaggcatcaaaaacacactgattgttgatgcggcaggctggggacaattttcccaatcaattgttgattatggccaaagcgtttttgcagcagatagcttaaaaaatacagtctttagcatccatatgtacgaatacgctggaaaagatgcagcaacagttaaagcgaatatggaaaacgtcctgaataaaggcctggcactgattattggcgaatttggcccgtatcatgtgaatggcgacgttgatgaactggcgattatgagatatggccaagaattgggcgttggctggcttgcatggtcatggtatggaaattcagacggccttcggtatctggatatggcaacaggaccgaatggatcactgacatcatttggcaatacagtcgtcaatgatacgtatggaatcaaaaatacgagccagaaagctggcatctttcagtaa

SEQ ID NO: 123 - DNA, 897 bp, artificial sequence
  nucleic acid sequence coding for PSpMan variant
gtggcgacaggcttttatgtttcaggcaataaactgtatgatagcacaggcaaagagtttgttatgagaggcgttaatcatggccatacctggtttaaaaacgatctgaatgaggcgattccggctattgcaaaaacaggcgcaaatacagttagaattgttctgtcaaatggcagcctgtatgagaaagatgatctggacgcagtcaaagacatcatcaatgtcgtcaacgataacaaaatgatagcagttctggaagttcatgatgcaacgggcaaagatgattacgattcactggatgcagcagtcaactattggatctcaattaaagaagcgctgatcggcaaagaagatcgcgttattgttaatattgcgaacgaatggatgggcacatggaatggctcagcatgggcagatggctacaaaagagcaattccgaaactgagaaatgcaggcatcaaaaacacactgattgttgatgcggcaggctggggacaatattcccaatcaattgttgattatggccaaagcgtttttgcagcagatagcttgaaaaatacagtctttagcatccatatgtacgaatacgctggaaaagatgcagcaacagttaaagcgaatatggaaaacgtcctgaataaaggcctggcactgattattggcgaatttggctgctatcatacaaatggcgacgttgatgaactggcgattatgagatatggccaagaattgggcgttggctggcttgcatggtcatggtatggaaattcagacggccttcggtatctggatatggcaacaggaccgaatggatcactgacatcatttggcaatacagtcgtcaatgatgcatatggaatcaaaaatacgagccagaaagctggcatctttcagtaa

SEQ ID NO: 124 - DNA, 897 bp, artificial sequence
  nucleic acid sequence coding for PSpMan variant
atggcgacaggctttgaagtttcaggcaccaaactgtatgatagcacaggcaaagagtttgttatgagaggcgttaatcattcccatacctggtttaaaaacgatctgaatgaggcgattccggctattgcaaaaacaggcgcaaatacagttagaattgttctgtcaaatggcagcctgtatacgctggatgatctggacgcagtcaaagacatcatcaatgtcgtcaaccagaacaaaatgatagcagttctggaagttcatgatgcaacgggcaaagatgattacgattcactggatgcagcagtcaactattggatctcaattaaaagcgcgctgatcggcaaagaagatcgcgttattgttaatattgcgaacgaatggatgggcacatggaatggcctggcatgggcagatggctacaaaaaagcaattccgaaactgagaaatgcaggcatcaaaaacacactgattgttgatgcggcaggctggggacaattttcccaatcaattgttgattatggccaaagcgtttttgcagcagatagcttgaaaaatacagtctttagcatccatatgtacgaatacgctggaaaagatgcagcaacagttaaagcgaatatggaaaacgtcctgaataaaggcctggcactgattattggcgaatttggctgctatcatgttaatggcgacgttgatgaactggcgattatgagatatggccaagaattgggcgttggctggcttgcatggtcatggtatggaaattcagacggccttcaatatctggatatggcaacaggaccgaatggatcactgacatcatttggcaatacagtcgtcaatagcacgtatggaatcaaaaatacgagccagaaagctggcatctttcagtaa

SEQ ID NO: 125 - DNA, 897 bp, artificial sequence
  nucleic acid sequence coding for PSpMan variant
atggcgacaggcttttatgtttcaggcaccaaactgtatgatagcacaggcaaagagtttgttatgagaggcgttaatcatggccatacctggtttaaaaacgatctgaatgaggcgattccggctattgcaaaaacaggcgcaaatacagttagaattgttctgtcaaatggcgtgcagtatacgagagatgatctggacgcagtcaaagatatcatcaatgtcgtcaaccagaacaaaatgattgcagttctggaagttcatgatgcaacgggcaaagatgattacgattcactggatgcagcaatcaactattggatctcaattaaagaagcgctgatcggcaaagaagatcgcgttattgttaatattgcgaacgaatggatgggcacatggaatggctcagcatgggcagatggctacaaacaggcaattccgaaactgagaaatgcaggcatcaaaaacacactgattgttgatgcggcaggctggggacaattttcccaatcaattgttgattatggccaaagcgtttttgcagcagatagcttaaaaaatacagtctttagcatccatatgtacgaatacgctggaaaagatgcagcaacagttaaagcgaatatggaaaacgtcctgaataaaggcctggcactgattattggcgaatttggcccgtatcatgtgaatggcgacgttgatgaactggcgattatgagatatggccaagaattgggcgttggctggcttgcatggtcatggtatggaaattcagacggccttcggtatctggatatggcaacaggaccgaatggatcactgacatcatttggcaatacagtcgtcaatgatacgtatggaatcaaaaatacgagccagaaagctggcatctttcagtaa

SEQ ID NO: 126 - DNA, 897 bp, artificial sequence
  nucleic acid sequence coding for PSpMan variant
atgtcaacaggcttttatgtttcaggcaataaactgtatgatagcacaggcaaagagtttgttatgagaggcgttaatcattcccatacctggtttaaaaacgatctgaatgaggcgattccggctattgcaaaaacaggcgcaaatacagttagaattgttctgtcaaatggcagcctgtatacgagagatgatctggacgcagtcaaagacatcatcgaagtcgtcaaccagaacaaaatgatagcagttctggaagttcatgatgcaacgggcagagatgattacgattcactggatgcagcagtcaactattggatctcaattaaagaagcgctgatcggcaaagaagatcgcgttattgttaatattgcgaacgaatggatgggcacatggaatggctcagcatgggcagatggctacaaaaaagcaattccgaaactgagaacagcaggcatcaagaacacactgattgttgatgcggcaggctggggacaattttcccaatcaattgttgattatggccaaagcgtttttgcagcagatagcttgaaaaatacagtctttagcatccatatgtacgaatacgctggaaaagatgcagcaacagttaaagcgaatatggaaaacgtcctggcaaaaggcctggcactgattattggcgaatttggctgctatcatacaaatggcgacgttgatgaactggcgattatgagatatggccaagaattgggcgttggctggcttgcatggtcatggtatggaaattcagacggccttcaatatctggatatggcaacaggaccgaatggatcactgacatcatttggcaatacagtcgtcaatgatacgtatggaatcaaaaatacgagccagaaagctggcatctttcagtaa

SEQ ID NO: 127 - DNA, 897 bp, artificial sequence
  nucleic acid sequence coding for PSpMan variant
ctggcgacaggcttttatgtttcaggcaccaaactgtatgatagcacaggcaaagagtttgttatgagaggcgttaatcatgcgcatacctggtttaaaaacgatctgaatgaggcgattccggctattgcaaaaacaggcgcaaatacagttagaattgttctgtcaaatggcagcctgtatacgctggatgatctggacgcagtcaaagacatcatcaatgtcgtcaacgataacaaaatgatagcagttctggaagttcatgatgcaacgggcaaagatgattacgattcactggatgcagcagtcaactattggatctcaattaaagaagcgctgatcggcaaagaagatcgcgttattgttaatattgcgaacgaatggatgggcacatggaatggctcactgtgggcagatggctacaaaaaagcaattccgaaactgagaaatgcaggcatcaaaaacacactgattgttgatgcggcaggctggggacaatttgcacaatcaattgttgattatggccaaagcgtttttgcagcagatagcttgaaaaatacagtctttagcatccatatgtacgaatacgctggaaaagatgcagcaacagttaaagcgaatatggaaaacgtcctggcaaaaggcctggcactgattattggcgaatttggctgctatcatacaaatggcgacgttgatgaactggcgattatgagatatggccaagaattgggcgttggctggcttgcatggtcatggtatggaaattcagacggccttcggtatctggatatggcaacaggaccgaatggatcactgacatcatttggcaatacagtcgtcaatgatacgtatggaatcaaaaatacgagccagaaagctggcatctttcagtaa

SEQ ID NO: 128 - DNA, 897 bp, artificial sequence
  nucleic acid sequence coding for PSpMan variant
atggcgacaggcttttatgtttcaggcaacaaactgtatgatagcacaggcaaagagtttgttatgagaggcgttaatcatggccatagctggtttaaaaacgatctgaatgaggcgattccggctattgcaaaaacaggcgcaaatacagttagaattgttctgtcaaatggcgtgctgtatacgagagatgatctggacgcagtcaaaaacatcatcaatgtcgtcaaccagaacaaaatgatagcagttctggaagttcatgatgcaacgggcaaagatgattacgattcactggatgcagcaatcaactattggatctcaattaaagaagcgctgatcggcaaagaagatcgcgttattgttaatattgcgaacgaatggatgggcacatggaatggctcagcatgggcagatggctacaaaaaagcaattccgaaactgagaaatgcaggcatcaaaaacacactgattgttgatgcggcaggctggggacaatatccgcaatcaattgttgattatggccaaagcgtttttgcagcagatagcttaaaaaatacagtctttagcatccatatgtacgaatacgctggaaaggatgcagcaacagttaaagcgaatatggaaaacgtcctgaataaaggcctggcactgattattggcgaatttggctgctatcatgtgaatggcgacgttgatgaactggcgattatgagatatggccaagaattgggcgttggctggcttgcatggtcatggtatggaaattcagacggccttcggtatctggatatggcaacaggaccgaatggatcactgacatcatttggcaatacagtcgtcaatgatacgtatggaatcaaaaatacgagccagaaagctggcatctttcagtaa

SEQ ID NO: 129 - DNA, 897 bp, artificial sequence
  nucleic acid sequence coding for PSpMan variant
atggcgacaggcttttatgtttcaggcaccaaactgtatgatagcacaggcaaagagtttgttatgagaggcgttaatcatgcgcatacctggtttaaaaacgatctgaatgaggcgattccggctattgcaaaaacaggcgcaaatacagttagaattgttctgtcaaatggcagcctgtatacgagagatgatctggacgcagtcaaaaacatcatcaatgtcgtcaaccagaacaaaatgatagcagttctggaagttcatgatgcaacgggcaaagatgattacgattcactggatgcagcagtcaactattggatctcaattaaagaagcgctgatcggcaaagaagatcgcgttattgttaatattgcgaacgaatggatgggcacatggaatggctcagcatgggcagatggctacaaaaaagcaattccgaaactgagaaatgcaggcatcaaaaacacactgattgttgatgcggcaggctggggacaatttccgcaatcaattgttgattatggccaaagcgtttttgcagcagatagcttgaaaaatacagtctttagcatccatatgtacgaatacgctggaaaagatgcagcaacagttaaagcgaatatggaaaacgtcctgaataaaggcctggcactgattattggcgaatttggctgctatcatgttaatggcgacgttgatgaactggcgattatgagatatggccaagaattgggcgttggctggcttgcatggtcatggtatggaaattcagacggccttcggtatctggatatggcaacaggaccgaatggatcactgacatcatttggcaatacagtcgtcaatgatacgtatggaatcaaaaatacgagccagaaagctggcatctttcagtaa

SEQ ID NO: 130 - DNA, 897 bp, artificial sequence
  nucleic acid sequence coding for PSpMan variant
atggcgagaggcttttatgtttcaggcaccaaactgtatgatagcacaggcaaagagtttgttatgagaggcgttaatcatgcgcatacctggtttaaaaacgatctgaatgaggcgattccggctattgcaaaaacaggcgcaaatacagttagaattgttctgtcaaatggcagcctgtatgagaaagatgatctggacgcagtcaaagacatcatcaatgtcgtcaaccagaacaaaatgatagcagttctggaagttcatgatgcaacgggcagagatgattacctgtcactggatgcagcagtcaactattggatctcaattaaaagcgcgctgatcggcaaagaagatcgcgttattgttaatattgcgaacgaatggatgggcacatggaatggctcagcatgggcaatgggctacaaaaaagcaattccgaaactgagaaatgcaggcatcaaaaacacactgattgttgatgcggcaggctggggacaattttcccaatcaattgttgattatggccaaagcgtttttgcagcagatagcttgaaaaatacagtctttagcatccatatgtacgaatacgctggaaaagatgcagcaacagttaaagcgaatatggaaaacgtcctgaataaaggcctggcactgattattggcgaatttggctgctatcatacaaatggcgacgttgatgaactggcgattatgagatatggccaagaattgggcgttggctggcttgcatggtcatggtatggaaattcagacggccttcaatatctggatatggcaacaggaccgaatggatcactgacatcatttggcaatacagtcgtcaatgatacgtatggaatcaaaaatacgagccagaaagctggcatctttcagtaa

SEQ ID NO: 131 - DNA, 897 bp, artificial sequence
  nucleic acid sequence coding for PSpMan variant
atggcgacaggcttttatgtttcaggcaccaaactgtatgatagcacaggcaaagagtttgttatgagaggcgttaatcatgcgcatacctggtttaaaaacgatctgaatgaggcgattccggctattgcaaaaacaggcgcaaatacagttagaattgttctgtcaaatggcgatctgtatacgaaagatgatctggactcagtcaaagacatcatcaatgtcgtcaaccagaacaaaatgatagcagttctggaagttcatgatgcaacgggcagagatgattacgattcactggatgcagcagtcaactattggatctcaataaaagaagcgctgatcggcaaagaagatcgcgttattgttaatattgcgaacgaatggatgggcacatggaatggctcagcatgggcagatggctacaaacaagcaattccgaaactgagaaatgcaggcatcaaaaacacactgattgttgatgcggcaggctggggacaattttcccaatcaattgttgattatggccaaagcgtttttgcagcagatagcgataaaaatacagtctttagcatccatatgtacgaatacgctggaaaagatgcagcaacagttaaagcgaatatggaaaacgtcctgaataaaggcctggcactgattattggcgaatttggctgctatcatacaaatggcgacgttgatgaactggcgattatgagatatggccaagaattgggcgttggctggcttgcatggtcatggtatggaaattcagacggccttcggtatctggatatggcaacaggaccgaatggatcactgacatcatttggcaatacagtcgtcaatgatgaatatggaatcaaaaatacgagccagaaagctggcatctttcagtaa

SEQ ID NO: 132 - DNA, 894 bp, artificial sequence
  nucleic acid sequence coding for PSpMan variant
atggcgacaggcttttatgtttcaggcaacaaactgtatgatagcacaggcaaagagtttgttatgagaggcgttaatcatggccatagctggtttaaaaacgatctgaatacagcgattccggctattgcaaaaacaggcgcaaatacagttagaattgttctgtcaaatggcagcctgtatacgctggatgatctgaatgcagtcaaagacatcatcaatgtcgtcaaccagaacaaaatgattgcagttctggaagttcatgatgcaacgggcaaagatgattacaattcactggatgcagcagtcaactattggatctcaattaaagaagcgctgatcggcaaggaagatcgcgttattgttaatattgcgaacgaatggatgggcacatggaatggctcagcatgggcagatggctacaaaaaagcaattccgaaactgagaaatgcaggcatcaaaaacacactgattgttgatgcggcaggctggggacaattttcccaatcaattgttgattatggccaaagcgtttttgcagcagatagcttgaaaaatacagtctttagcatccatatgtacgaatacgctggaaaagatgcagcaacagtcaaagcgaatatggaaaacgtcctgaataaaggcctggcactgattattggcgaatttggctgctatcatacaaatggcgacgttgatgaatatgcgattatgagatatggccaagaattgggcgttggctggcttgcatggtcatggtatggaaattcatcacgccttaactatctagatatggcaacaggaccgaatggatcactgacatcatttggcaatacagtcgtcaatgatacgtatggaatcaaaaatacgagccagaaagctggcatcttttaa

SEQ ID NO: 133 - DNA, 894 bp, artificial sequence
  nucleic acid sequence coding for PSpMan variant
atggcgacaggcttttatgtttcaggcaacaaactgtatgatagcacaggcaaagagtttgttatgagaggcgttaatcatggccatagctggtttaaaaacgatctgaatacagcgattccggctattgcaaaaacaggcgcaaatacagttagaattgttctgtcaaatggcagcctgtatacgaaagatgatctggacgcagtcaaagacatcatcaatgtcgtcaacgacaacacgatgattgcagttctggaagttcatgatgcaacgggcaaagatgattacgattcactggatgcagcagtcaactattggatctcaattaaagaagcgctgatcggcaaagaagatcgcgttattgttaatattgcgaacgaatggatgggcacatggaatggctcagcatgggcagatggctacaaaaaagcaattccgaaactgagaaatgcaggcatcaaaaacacactgattgttgatgcggcaggctggggacaattttcccaatcaattgttgattatggccaaagcgtttttgcagcagatagcttgaaaaatacagtctttagcatccatatgtacgaatacgctggaaaagatgcagcaacagttaaagcgaatatggaaaacgtcctgaataaaggcctggcactgattattggcgaatttggcggatatcatacaaatggcgacgttgatgaatatgcgattatgagatatggccaagaattgggcgttggctggcttgcatggtcatggtatggaaattcatcaggccttaactatctcgatatggcaacaggaccgaatggatcactgacatcatttggcaatacagtcgtcaatgatacgtatggaatcaaaaatacgagccagaaagctggcatcttttaa

SEQ ID NO: 134 - DNA, 894 bp, artificial sequence
  nucleic acid sequence coding for PSpMan variant
atggcgacaggcttttatgtttcaggcaacaaactgtatgatagcacaggcaaagagtttgttatgaggggcgttaatcatggccatagctggtttaaaaacgatctgaatgaggcgattccggctattgcaaaaacaggcgcaaatacagttagaattgttctgtcaaatggcagcctgtatacgaaagatgatctggacgcagtcaaaaacatcatcaatgtcgtcaaccagaacaaaatgattgcagttctggaagttcatgatgcaacgggcaaagatgattacaattcactggatgcagcagtcaactattggatctcaattaaagaagcgctgatcggcaaagaagatcgcgtcattgttaatattgcgaacgaatggatgggcacatggaatggctcagcatgggcagatggctacaaaaaagcaattccgaaactgagaaatgcaggcatcaaaaacacactgattgttgatgcggcaggctggggacaattttcccaatcaattgttgattatggccaaagcgtttttgcagcagatagcttgaaaaatacagtctttagcatccatatgtacgaatacgctggaaaagatgcagcaacagttaaagcgaatatggaaaacgtcctgaataaaggcctggcactgattattggcgaatttggcggatatcatgtgaatggcgacgttgatgaatatgcgattatgagatatggccaagaattgggcgttggctggcttgcatggtcatggtatggaaattcatcaggccttaactatctggatatggcaacaggaccgaatggatcactgacatcatttggcaatacagtcgtcaatgatacgtatggaatcaaaaatacgagccagaaagctggcatcttttaa

SEQ ID NO: 135 - DNA, 894 bp, artificial sequence
  nucleic acid sequence coding for PSpMan variant
atggcgacaggcttttatgtttcaggcaacaaactgtatgatagcacaggcaaagagtttgttatgagaggcgttaatcatggccatagctggtttaaaaacgatctgaatgaggcgattccggctattgcaaaaacaggcgcaaatacagttagaattgttctgtcaaatggcagcctgtatacgaaagatgatctggacgcagtcaaaaacatcatcaatgtcgtcaaccagaacaaaatgattgcagttctggaagttcatgatgcaacgggcaaagatgattacaattcactggatgcagcagtcaactattggatctcaattaaagaagcgctgatcggcaaagaagatcgcgttattgttaatattgcgaacgaatggatgggcacatggaatggctcagcatgggcagatggctacaaaaaagcaattccgaaactgagaaatgcaggcatcaaaaacacactgattgttgatgcggcaggctggggacaatttccgcaatcaattgttgattatggccaaagcgtttttgcagcagatagcttgaaaaatacagtctttagcatccatatgtacgaatacgctggaaaagatgcagcaacagttaaagcgaatatggaaaacgtcctgaataaaggcctggcactgattattggcgaatttggcggatatcatacaaatggcgacgttgatgaatatgcgattatgagatatggccaagaactgggcgttggctggcttgcatggtcatggtatggaaattcagacggccttcggtatctggatatggcaacaggaccgaatggatcactgacatcatttggcaatacagtcgtcaatgatacgtatggaatcaaaaatacgagccagaaagctggcatcttttaa

SEQ ID NO: 136 - DNA, 894 bp, artificial sequence
  nucleic acid sequence coding for PSpMan variant
atggcgacaggcttttatgtttcaggcaacaaactgtatgatagcacaggcaaagagtttgttatgaggggcgttaatcatggccatagctggtttaaaaacgatctgaatacagcgattccggctattgcaaaaacaggcgcaaatacagttagaattgttctgtcaaatggcagcctgtatacgctggatgatctgaatgcagtcaaagacatcatcaatgtcgtcaaccagaacaaaatgattgcagttctggaagttcatgatgcaacgggcaaagatgattacaattcactggatgcagcagtcaactattggatctcaattaaagaagcgctgatcggcaaagaagatcgcgttattgttaatattgcgaacgaatggatgggcacatggaatggctcagcatgggcagatggctacaaaaaagcaattccgaaactgagaaatgcaggcatcaaaaacacactgattgttgatgcggcaggctggggacaattttcccaatcaattgttgattatggccaaagcgtttttgcagcagatagcttgaaaaatacagtctttagcatccatatgtacgaatacgctggaaaagatgcagcaacagtcaaagcgaatatggaaaacgtcctgaataaaggcctggcactgattattggcgaatttggcggatatcatacaaatggcgacgttgatgaatatgcgattatgagatatggccaagaattgggcgttggctggcttgcatggtcatggtatggaaattcagacggccttcggtatctggatatggcaacaggaccgaatggatcactgacatcatttggcaatacagtcgtcaatgatacgtatggaatcaaaaatacgagccagaaagctggcatcttttaa

SEQ ID NO: 137 - DNA, 894 bp, artificial sequence
  nucleic acid sequence coding for PSpMan variant
atggcgacaggcttttatgtttcaggcaacaaactgtatgatagcacaggcaaagagtttgttatgaggggcgttaatcatggccatagctggtttaaaaacgatctgaatgaggcgattccggctattgcaaaaacaggcgcaaatacagttagaattgttctgtcaaatggcagcctgtatacgctggatgatctgaatgcagtcaaagacatcatcaatgtcgtcaaccagaacaaaatgattgcagttctggaagttcatgatgcaacgggcaaagatgattacaattcactggatgcagcagtcaactattggatctcaattaaagaagcgctgatcggcaaagaagatcgcgttattgttaatattgcgaacgaatggatgggcacatggaatggctcagcatgggcagatggctacaaaaaagcaattccgaaactgagaaatgcaggcatcaaaaacacactgattgttgatgcggcaggctgggggcagttttcccaatcaattgttgattatggccaaagcgtttttgcagcagatagcttgaaaaatacagtctttagcatccatatgtacgaatacgctggaaaagatgcagcaacagttaaagcgaatatggaaaacgtcctgaataaaggcctggcactgattattggcgaatttggcggatatcatacaaatggcgacgttgatgaatatgcgattatgagatatggccaagaattgggcgttggctggcttgcatggtcatggtatggaaattcagacccccttaactatctggatatggcaacaggaccgaatggatcactgacatcatttggcaatacagtcgtcaatgatacgtatggaatcaaaaatacgagccagaaagctggcatcttttaa

SEQ ID NO: 138 - DNA, 894 bp, artificial sequence
  nucleic acid sequence coding for PSpMan variant
atggcgacaggcttttatgtttcaggcaacaaactgtatgatagcacaggcaaaccgtttgttatgagaggcgttaatcatggccatagctggtttaaaaacgatctgaatacagcgattccggctattgcaaaaacaggcgcaaatacagttagaattgttctgtcaaatggcagcctgtatacgctggatgatctgaatgcagtcaaagacatcatcaatgtcgtcaaccagaacaaaatgattgcagttctggaagttcatgatgcaacgggcaaagatgattacaattcactggatgcagcagtcaactattggatctcaattaaagaagcgctgatcggcaaagaagatcgcgttattgttaatattgcgaacgaatggatgggcacatggaatggctcagcatgggcagatggctacaaaagagcaattccgaaactgagaaatgcaggcatcaaaaacacactgattgttgatgcggcaggctggggacaattttcccaatcaattgttgattatggccaaagcgtttttgcagcagatagcttgaaaaatacagtctttagcatccatatgtacgaatacgctggaaaagatgcagcaacagttaaagcgaatatggaaaacgtcctgaataaaggcctggcactgattattggcgaatttggctgctatcatgtgaatggcgacgttgatgaatatgcgattatgagatatggccaagaattgggcgttggctggcttgcatggtcatggtatggaaattcagacccccttaactatctggatatggcaacaggaccgaatggatcactgacatcatttggcaatacagtcgtcaatgatacgtatggaatcaaaaatacgagccagaaagctggcatcttctaa

SEQ ID NO: 139 - DNA, 894 bp, artificial sequence
  nucleic acid sequence coding for PSpMan variant
atggcgacaggcttttatgtttcaggcaacaaactgtatgatagcacaggcaaagagtttgttatgagaggcgttaatcatggccatagctggtttaaaaacgatctgaatgaggcgattccggctattgcaaaaacaggcgcaaatacagttagaattgttctgtcaaatggcagcctgtatacgctggatgatctgaatgcagtcaaagacatcatcaatgtcgtcaaccagaacaaaatgattgcagttctggaagttcatgatgcaacgggcaaagatgattacaattcactggatgcagcagtcaactattggatctcaattaaagaagcgctgatcggcaaagaagatcgcgttattgttaatattgcgaacgaatggatgggcacatggaatggctcagcatgggcagatggctacaaaaaagcaattccgaaactgagaaatgcaggcatcaaaaacacactgattgttgatgcggcaggctggggacaattttcccaatcaattgttgattatggccaaagcgtttttgcagcagatagcttgaaaaatacagtctttagcatccatatgtacgaatacgctggaaaagatgcagcaacagttaaagcgaatatggaaaacgtcctgaataaaggcctggcactgattattggcgaatttggcggatatcatacaaatggcgacgttgatgaatatgcgattatgagatatggccaagaactgggcgttggctggcttgcatggtcatggtatggaaattcagacggccttcggtatctggatatggcaacaggaccgaatggatcactgacatcatttggcaatacagtcgtcaatgatacgtatggaatcaaaaatacgagccagaaagctggcatcttttaa

SEQ ID NO: 140 - protein, 29 aa, artificial sequence
  synthetic
VRSKKLWISLLFALTLIFTMAFSNMSAQA

SEQ ID NO: 141 - protein, 297 aa, artificial sequence
  PspMan variant
MATGFYVSGNKLYDSTGKPFVMRGVNHGHSWFKNDLNTAIPAIAKTGANTVRIVLSNGSLYTKDDLNAVKNIINVVNQNKMIAVLEVHDATGKDDYNSLDAAVNYWISIKEALIGKEDRVIVNIANEWMGTWNGSAWADGYKKAIPKLRNAGIKNTLIVDAAGWGQFPQSIVDYGQSVFAADSQKNTVFSIHMYEYAGKDAATVKANMENVLNKGLALIIGEFGGYHTNGDVDEYAIMRYGQELGVGWLAWSWYGNSSGLNYLDMATGPNGSLTSFGNTVVNDTYGIKNTSQKAGIF

SEQ ID NO: 142 - protein, 297 aa, artificial sequence
  PspMan variant
MATGFYVSGNKLYDSTGKPFVMRGVNHGHSWFKNDLNTAIPAIAKTGANTVRIVLSNGSLYTKDDLNAVKNIINVVNQNKMIAVLEVHDATGKDDYNSLDAAVNYWISIKEALIGKEDRVIVNIANEWMGTWNGSAWADGYKQAIPKLRNAGIKNTLIVDAAGWGQFPQSIVDYGQSVFAADSQKNTVFSIHMYEYAGKDAATVKANMENVLNKGLALIIGEFGGYHTNGDVDEYAIMRYGQELGVGWLAWSWYGNSSGLNYLDMATGPNGSLTSFGNTVVNDTYGIKNTSQKAGIF

SEQ ID NO: 143 - protein, 297 aa, artificial sequence
  PspMan variant
MATGFYVSGNKLYDSTGKPFVMRGVNHGHSWFKNDLNEAIPAIAKTGANTVRIVLSNGSLYTKDDLNAVKNIINVVNQNKMIAVLEVHDATGKDDYNSLDAAVNYWISIKEALIGKEDRVIVNIANEWYGTWNGSAWADGYKKAIPKLRNAGIKNTLIVDAAGWGQFPQSIVDYGQSVFAADSQKNTVFSIHMYEYAGKDAATVKANMENVLNKGLALIIGEFGGYHTNGDVDEYAIMRYGQEKGVGWLAWSWYGNSDGLNYLDMATGPNGSLTSFGNTVVNDTYGIKNTSQKAGIF

SEQ ID NO: 144 - protein, 297 aa, artificial sequence
  PspMan variant
MATGFYVSGNKLYDSTGKPFVMRGVNHGHSWFKNDLNEAIPAIAKTGANTVRIVLSNGSLYTKDDLNAVKNIINVVNQNKMIAVLEVHDATGKDDYNSLDAAVNYWISIKEALIGKEDRVIVNIANEWYGTWNGSAWADGYKQAIPKLRNAGIKNTLIVDAAGWGQFPQSIVDYGQSVFAADSQKNTVFSIHMYEYAGKDAATVKANMENVLNKGLALIIGEFGGYHTNGDVDEYAIMRYGQEKGVGWLAWSWYGNSDGLNYLDMATGPNGSLTSFGNTVVNDTYGIKNTSQKAGIF

SEQ ID NO: 145 - protein, 297 aa, artificial sequence
  PspMan variant
MATGFYVSGNKLYDSTGKEFVMRGVNHGHSWFKNDLNTAIPAIAKTGANTVRIVLSNGSLYTKDDLNAVKNIINVVNQNKMIAVLEVHDATGKDDYNSLDAAVNYWISIKEALIGKEDRVIVNIANEWYGTWNGSAWADGYKKAIPKLRNAGIKNTLIVDAAGWGQFPQSIVDYGQSVFAADSDKNTVFSIHMYEYAGKDAATVKANMENVLNKGLALIIGEFGGYHTNGDVDEYAIMRYGQEKGVGWLAWSWYGNSSGLNYLDMATGPNGSLTSFGNTVVNDTYGIKNTSQKAGIF

SEQ ID NO: 146 - protein, 297 aa, artificial sequence
  PspMan variant
MATGFYVSGNKLYDSTGKEFVMRGVNHGHSWFKNDLNTAIPAIAKTGANTVRIVLSNGSLYTKDDLNAVKNIINVVNQNKMIAVLEVHDATGKDDYNSLDAAVNYWISIKEALIGKEDRVIVNIANEWYGTWNGSAWADGYKQAIPKLRNAGIKNTLIVDAAGWGQFPQSIVDYGQSVFAADSDKNTVFSIHMYEYAGKDAATVKANMENVLNKGLALIIGEFGGYHTNGDVDEYAIMRYGQEKGVGWLAWSWYGNSSGLNYLDMATGPNGSLTSFGNTVVNDTYGIKNTSQKAGIF

SEQ ID NO: 147 - protein, 297 aa, artificial sequence
  PspMan variant
MATGFYVSGNKLYDSTGKEFVMRGVNHGHSWFKNDLNTAIPAIAKTGANTVRIVLSNGSLYTKDDLNAVKNIINVVNQNKMIAVLEVHDATGKDDYNSLDAAVNYWISIKEALIGKEDRVIVNIANEWYGTWNGSAWADGYKKAIPKLRNAGIKNTLIVDAAGWGQFPQSIVDYGQSVFAADSLKNTVFSIHMYEYAGKDAATVKANMENVLNKGLALIIGEFGGYHTNGDVDEYAIMRYGQEKGVGWLAWSWYGNSSGLNYLDMATGPNGSLTSFGNTVVNDTYGIKNTSQKAGIF

SEQ ID NO: 148 - protein, 297 aa, artificial sequence
  PspMan variant
MATGFYVSGNKLYDSTGKEFVMRGVNHGHSWFKNDLNTAIPAIAKTGANTVRIVLSNGSLYTKDDLNAVKNIINVVNQNKMIAVLEVHDATGKDDYNSLDAAVNYWISIKEALIGKEDRVIVNIANEWYGTWNGSAWADGYKQAIPKLRNAGIKNTLIVDAAGWGQFPQSIVDYGQSVFAADSLKNTVFSIHMYEYAGKDAATVKANMENVLNKGLALIIGEFGGYHTNGDVDEYAIMRYGQEKGVGWLAWSWYGNSSGLNYLDMATGPNGSLTSFGNTVVNDTYGIKNTSQKAGIF

SEQ ID NO: 149 - protein, 297 aa, artificial sequence
  PspMan variant
MATGFYVSGNKLYDSTGKPFVMRGVNHGHSWFKNDLNTAIPAIAKTGANTVRIVLSNGSLYTKDDLNAVKNIINVVNQNKMIAVLEVHDATGKDDYDSLDAAVNYWISIKEALIGKEDRVIVNIANEWYGTWNGSAWADGYKKAIPKLRNAGIKNTLIVDAAGWGQFPQSIVDYGQSVFAADSQKNTVFSIHMYEYAGKDAATVKANMENVLNKGLALIIGEFGCYHTNGDVDEYAIMRYGQEKGVGWLAWSWYGNSSGLNYLDMATGPNGSLTSFGNTVVNDTYGIKNTSQKAGIF

SEQ ID NO: 150 - protein, 297 aa, artificial sequence
  PspMan variant
MATGFYVSGNKLYDSTGKPFVMRGVNHGHSWFKNDLNTAIPAIAKTGANTVRIVLSNGSLYTKDDLNAVKNIINVVNQNKMIAVLEVHDATGKDDYDSLDAAVNYWISIKEALIGKEDRVIVNIANEWYGTWNGSAWADGYKQAIPKLRNAGIKNTLIVDAAGWGQFPQSIVDYGQSVFAADSQKNTVFSIHMYEYAGKDAATVKANMENVLNKGLALIIGEFGCYHTNGDVDEYAIMRYGQEKGVGWLAWSWYGNSSGLNYLDMATGPNGSLTSFGNTVVNDTYGIKNTSQKAGIF

SEQ ID NO: 151 - protein, 297 aa, artificial sequence
  PspMan variant
MATGFYVSGNKLYDSTGKPFVMRGVNHGHSWFKNDLNTAIPAIAKTGANTVRIVLSNGSLYTKDDLNAVKNIINVVNQNKMIAVLEVHDATGKDDYDSLDAAVNYWISIKEALIGKEDRVIVNIANEWYGTWNGSAWADGYKKAIPKLRNAGIKNTLIVDAAGWGQFPQSIVDYGQSVFAADSQKNTVFSIHMYEYAGKDAATVKANMENVLNKGLALIIGEFGPYHTNGDVDEYAIMRYGQEKGVGWLAWSWYGNSSGLNYLDMATGPNGSLTSFGNTVVNDTYGIKNTSQKAGIF

SEQ ID NO: 152 - protein, 297 aa, artificial sequence
  PspMan variant
MATGFYVSGNKLYDSTGKPFVMRGVNHGHSWFKNDLNTAIPAIAKTGANTVRIVLSNGSLYTKDDLNAVKNIINVVNQNKMIAVLEVHDATGKDDYDSLDAAVNYWISIKEALIGKEDRVIVNIANEWYGTWNGSAWADGYKQAIPKLRNAGIKNTLIVDAAGWGQFPQSIVDYGQSVFAADSQKNTVFSIHMYEYAGKDAATVKANMENVLNKGLALIIGEFGPYHTNGDVDEYAIMRYGQEKGVGWLAWSWYGNSSGLNYLDMATGPNGSLTSFGNTVVNDTYGIKNTSQKAGIF

SEQ ID NO: 153 - protein, 297 aa, artificial sequence
  PspMan variant
MATGFYVSGNKLYDSTGKPFVMRGVNHGHSWFKNDLNTAIPAIAKTGANTVRIVLSNGSLYTKDDLDAVKNIINVVNQNKMIAVLEVHDATGKDDYNSLDAAVNYWISIKEALIGKEDRVIVNIANEWYGTWNGSAWADGYKKAIPKLRNAGIKNTLIVDAAGWGQFSQSIVDYGQSVFAADSQKNTVFSIHMYEYAGKDAATVKANMENVLNKGLALIIGEFGGYHTNGDVDEYAIMRYGQEKGVGWLAWSWYGNSSGLNYLDMATGPNGSLTSFGNTVVNDTYGIKNTSQKAGIF

SEQ ID NO: 154 - protein, 297 aa, artificial sequence
  PspMan variant
MATGFYVSGNKLYDSTGKPFVMRGVNHGHSWFKNDLNTAIPAIAKTGANTVRIVLSNGSLYTKDDLDAVKNIINVVNQNKMIAVLEVHDATGKDDYNSLDAAVNYWISIKEALIGKEDRVIVNIANEWYGTWNGSAWADGYKQAIPKLRNAGIKNTLIVDAAGWGQFSQSIVDYGQSVFAADSQKNTVFSIHMYEYAGKDAATVKANMENVLNKGLALIIGEFGGYHTNGDVDEYAIMRYGQEKGVGWLAWSWYGNSSGLNYLDMATGPNGSLTSFGNTVVNDTYGIKNTSQKAGIF

SEQ ID NO: 155 - protein, 297 aa, artificial sequence
  PspMan variant
MATGFYVSGNKLYDSTGKPFVMRGVNHGHSWFKNDLNTAIPAIAKTGANTVRIVLSNGSLYTLDDLNAVKDIINVVNQNKMIAVLEVHDATGKDDYNSLDAAVNYWISIKEALIGKEDRVIVNIANEWYGTWNGSAWADGYKKAIPKLRNAGIKNTLIVDAAGWGQFPQSIVDYGQSVFAADSQKNTVFSIHMYEYAGKDAATVKANMENVLNKGLALIIGEFGGYHTNGDVDEYAIMRYGQEKGVGWLAWSWYGNSSGLNYLDMATGPNGSLTSFGNTVVNDTYGIKNTSQKAGIF

SEQ ID NO: 156 - protein, 297 aa, artificial sequence
  PspMan variant
MATGFYVSGNKLYDSTGKPFVMRGVNHGHSWFKNDLNTAIPAIAKTGANTVRIVLSNGSLYTLDDLNAVKDIINVVNQNKMIAVLEVHDATGKDDYNSLDAAVNYWISIKEALIGKEDRVIVNIANEWYGTWNGSAWADGYKQAIPKLRNAGIKNTLIVDAAGWGQFPQSIVDYGQSVFAADSQKNTVFSIHMYEYAGKDAATVKANMENVLNKGLALIIGEFGGYHTNGDVDEYAIMRYGQEKGVGWLAWSWYGNSSGLNYLDMATGPNGSLTSFGNTVVNDTYGIKNTSQKAGIF

SEQ ID NO: 157 - protein, 297 aa, artificial sequence
  PspMan variant
MATGFYVSGNKLYDSTGKPFVMRGVNHGHSWFKNDLNTAIPAIAKTGANTVRIVLSNGSLYTRDDLNAVKDIINVVNQNKMIAVLEVHDATGKDDYNSLDAAVNYWISIKEALIGKEDRVIVNIANEWYGTWNGSAWADGYKKAIPKLRNAGIKNTLIVDAAGWGQFPQSIVDYGQSVFAADSQKNTVFSIHMYEYAGKDAATVKANMENVLNKGLALIIGEFGGYHTNGDVDEYAIMRYGQEKGVGWLAWSWYGNSSGLNYLDMATGPNGSLTSFGNTVVNDTYGIKNTSQKAGIF

SEQ ID NO: 158 - protein, 297 aa, artificial sequence
  PspMan variant
MATGFYVSGNKLYDSTGKPFVMRGVNHGHSWFKNDLNTAIPAIAKTGANTVRIVLSNGSLYTKDDLNAVKNIINVVNQNKMIAVLEVHDATGKDDYNSLDAAVNYWISIKEALIGKEDRVIVNIANEWYGTWNGSAWADGYKKAIPKLRNAGIKNTLIVDAAGWGQFPQSIVDYGQSVFAADSQKNTVFSIHMYEYAGKDAATVKANMENVLNKGLALIIGEFGGYHVNGDVDELAIMRYGQEKGVGWLAWSWYGNSSGLNYLDMATGPNGSLTSFGNTVVNDTYGIKNTSQKAGIF

SEQ ID NO: 159 - protein, 297 aa, artificial sequence
  PspMan variant
MATGFYVSGNKLYDSTGKPFVMRGVNHGHSWFKNDLNTAIPAIAKTGANTVRIVLSNGSLYTKDDLNAVKNIINVVNQNKMIAVLEVHDATGKDDYNSLDAAVNYWISIKEALIGKEDRVIVNIANEWYGTWNGSAWADGYKQAIPKLRNAGIKNTLIVDAAGWGQFPQSIVDYGQSVFAADSQKNTVFSIHMYEYAGKDAATVKANMENVLNKGLALIIGEFGGYHVNGDVDELAIMRYGQEKGVGWLAWSWYGNSSGLNYLDMATGPNGSLTSFGNTVVNDTYGIKNTSQKAGIF

SEQ ID NO: 160 - protein, 299 aa, unknown
  Bacillus sp.
ANSGFYVSGTTLYDANGNPFVMRGINHGHAWYKDQATTAIEGIANTGANTVRIVLSDGGQWTKDDIHTVRNLISLAEDNHLVAVPEVHDATGYDSIASLNRAVDYWIEMRSALIGKEDTVIINIANEWFGSWEGDAWADGYKQAIPRLRNAGLNHTLMVDAAGWGQFPQSIHDYGREVFNADPQRNTMFSIHMYEYAGGNASQVRTNIDRVLNQDLALVIGEFGHRHTNGDVDEATIMSYSEQRGVGWLAWSWKGNGPEWEYLDLSNDWAGNNLTAWGNTIVNGPYGLRETSRLSTVFT

SEQ ID NO: 161 - protein, 297 aa, artificial sequence
  PspMan variant
MATGFYVSGNKLYDSTGKPFVMRGVNHGHSWFKNDLNTAIPAIAKTGANTVRIVLSNGSQWTKDDLNAVKNIINVVNQNKMIAVLEVHDATGKDDYNSLDAAVNYWISIKEALIGKEDRVIVNIANEWYGTWNGSAWADGYKKAIPKLRNAGIKNTLIVDAAGWGQFPQSIVDYGQSVFAADSQKNTVFSIHMYEYAGKDAATVKANMENVLNKGLALIIGEFGGYHTNGDVDEYAIMRYGQEKGVGWLAWSWYGNSSGLNYLDMATGPNGSLTSFGNTVVNDTYGIKNTSQKAGIF

SEQ ID NO: 162 - protein, 309 aa, unknown
  Bacillus sp.
ANSGFYVSGTTLYDANGNPFVMRGINHGHAWYKDQATTAIEGIANTGANTVRIVLSDGGQWTKDDIHTVRNLISLAEDNHLVAVPEVHDATGYDSIASLNRAVDYWIEMRSALIGKEDTVIINIANEWFGSWEGDAWADGYKQAIPRLRNAGLNHTLMVDAAGWGQFPQSIHDYGREVFNADPQRNTMFSIHMYEYAGGNASQVRTNIDRVLNQDLALVIGEFGHRHTNGDVDEATIMSYSEQRGVGWLAWSWKGNGPEWEYLDLSNDWAGNNLTAWGNTIVNGPYGLRETSRLSTVFTGGGSDGGTSP